European Patent Application EP 4 516 806 A2, published March 5, 2025. Title: G PROTEINS. Applicant: Nxera Pharma UK Limited. The sequence listing filed with the application follows.

SEQUENCE LISTING (166 sequences)

SEQ ID NO: 1 - protein, 288 aa, synthetic construct
  REGION 1..288: note = MINI GS55
MGHHHHHHHHHHENLYFQSGCLGNSKTEDQRNEEKAQREANKKIEKQLQKDKQVYRATHRLLLLGAGESGKSTIVKQMRILHVNGGGDQDLLRCRVLTSGIFETKFQVDKVNFHMFDVGGQRDERRKWIQCFNDVTAIIFVVASSSYNMVIREDNQTNRLQEALNLFKSIWNNRWLRTISVILFLNKQDLLAEKVLAGKSKIEDYFPEFARYTTPEDATPEPGEDPRVTRAKYFIRDEFLRISTASGDGRHYCYPHFTCAVDTENIRRVFNDCRDIIQRMHLRQYELL

SEQ ID NO: 2 - protein, 257 aa, synthetic construct
  REGION 1..257: note = MINI GS77
MGHHHHHHANKKIEKQLQKDKQVYRATHRLLLLGAGESGKSTIVKQMRILHVNGGGDQDALRSRVLTSGIFETKFQVDKVNFHMFDVGGQRDERRKWIQCFNDVTAIIFVVASSSYNMVIREDNQTNRLQEALNLFKSIWNNRWLRTISVILFLNKQDLLAEKVLAGKSKIEDYFPEFARYTTPEDATPEPGEDPRVTRAKYFIRDEFLRISTASGDGRHYCYPHFTCAVDTENIRRVFNDCRDIIQRMHLRQYELL

SEQ ID NO: 3 - protein, 257 aa, synthetic construct
  REGION 1..257: note = MINI GS81
MGHHHHHHANKKIEKQLQKDKQVYRATIRLLLLGAGESGKSTIVKQMRILHVNGGGDQDALRSRVLTSGIFETKFQVDKVNFHMFDVGGQRDERRKWIQCFNDVTAIIFVVASSSYNMVIREDNQTNRLQEALNLFKSIWNNRWLRTISVILFLNKQDLLAEKVLAGKSKIEDYFPEFARYTTPEDATPEPGEDPRVTRAKYFIRDEFLRISTASGDGRHYCYPHFTCAVDTENIRRVFNDCRDIIQRMHLRQYELL

SEQ ID NO: 4 - protein, 257 aa, synthetic construct
  REGION 1..257: note = MINI GS84
MGHHHHHHANKKIEKQLQKDKQVYRATVRLLLLGAGESGKSTIVKQMRILHVNGGGDQDALRSRVLTSGIFETKFQVDKVNFHMFDVGGQRDERRKWIQCFNDVTAIIFVVASSSYNMVIREDNQTNRLQEALNLFKSIWNNRWLRTISVILFLNKQDLLAEKVLAGKSKIEDYFPEFARYTTPEDATPEPGEDPRVTRAKYFIRDEFLRISTASGDGRHYCYPHFTCAVDTENIRRVFNDCRDIIQRMHLRQYELL

SEQ ID NO: 5 - protein, 257 aa, synthetic construct
  REGION 1..257: note = MINI GS186
MGHHHHHHANKKIEKQLQKDKQVYRATHRLLLLGLGESGKSTIVKQMRILHVNGGGDQDALRSRVLTSGIFETKFQVDKVNFHMFDVGGQRDERRKWIQCFNDVTAIIFVVASSSYNMVIREDNQTNRLQEALNLFKSIWNNRWLRTISVILFLNKQDLLAEKVLAGKSKIEDYFPEFARYTTPEDATPEPGEDPRVTRAKYFIRDEFLRISTASGDGRHYCYPHFTCAVDTENIRRVFNDCRDIIQRMHLRQYELL

SEQ ID NO: 6 - protein, 257 aa, synthetic construct
  REGION 1..257: note = MINI GS130
MGHHHHHHANKKIEKQLQKDKQVYRATHRLLLLGADESGKSTIVKQMRILHVNGGGDQDALRSRVLTSGIFETKFQVDKVNFHMFDVGGQRDERRKWIQCFNDVTAIIFVVASSSYNMVIREDNQTNRLQEALNLFKSIWNNRWLRTISVILFLNKQDLLAEKVLAGKSKIEDYFPEFARYTTPEDATPEPGEDPRVTRAKYFIRDEFLRISTASGDGRHYCYPHFTCAVDTENIRRVFNDCRDIIQRMHLRQYELL

SEQ ID NO: 7 - protein, 257 aa, synthetic construct
  REGION 1..257: note = MINI GS116
MGHHHHHHANKKIEKQLQKDKQVYRATHRLLLLGAGNSGKSTIVKQMRILHVNGGGDQDALRSRVLTSGIFETKFQVDKVNFHMFDVGGQRDERRKWIQCFNDVTAIIFVVASSSYNMVIREDNQTNRLQEALNLFKSIWNNRWLRTISVILFLNKQDLLAEKVLAGKSKIEDYFPEFARYTTPEDATPEPGEDPRVTRAKYFIRDEFLRISTASGDGRHYCYPHFTCAVDTENIRRVFNDCRDIIQRMHLRQYELL

SEQ ID NO: 8 - protein, 257 aa, synthetic construct
  REGION 1..257: note = MINI GS134
MGHHHHHHANKKIEKQLQKDKQVYRATHRLLLLGAGESGKSTIVKQMRILHVNGGGDQDALRSAVLTSGIFETKFQVDKVNFHMFDVGGQRDERRKWIQCFNDVTAIIFVVASSSYNMVIREDNQTNRLQEALNLFKSIWNNRWLRTISVILFLNKQDLLAEKVLAGKSKIEDYFPEFARYTTPEDATPEPGEDPRVTRAKYFIRDEFLRISTASGDGRHYCYPHFTCAVDTENIRRVFNDCRDIIQRMHLRQYELL

SEQ ID NO: 9 - protein, 257 aa, synthetic construct
  REGION 1..257: note = MINI GS111
MGHHHHHHANKKIEKQLQKDKQVYRATHRLLLLGAGESGKSTIVKQMRILHVNGGGDQDALRSRVLTSGIFETKFQVDKVNFHMFDVGAQRDERRKWIQCFNDVTAIIFVVASSSYNMVIREDNQTNRLQEALNLFKSIWNNRWLRTISVILFLNKQDLLAEKVLAGKSKIEDYFPEFARYTTPEDATPEPGEDPRVTRAKYFIRDEFLRISTASGDGRHYCYPHFTCAVDTENIRRVFNDCRDIIQRMHLRQYELL

SEQ ID NO: 10 - protein, 255 aa, synthetic construct
  REGION 1..255: note = MINI GS98
MGHHHHHHANKKIEKQLQKDKQVYRATHRLLLLGAGESGKSTIVKQMRILHVNGGGDQDALRSRVLTSGIFETKFQVDKVNFHMFDVGGGGRRKWIQCFNDVTAIIFVVASSSYNMVIREDNQTNRLQEALNLFKSIWNNRWLRTISVILFLNKQDLLAEKVLAGKSKIEDYFPEFARYTTPEDATPEPGEDPRVTRAKYFIRDEFLRISTASGDGRHYCYPHFTCAVDTENIRRVFNDCRDIIQRMHLRQYELL

SEQ ID NO: 11 - protein, 257 aa, synthetic construct
  REGION 1..257: note = MINI GS175
MGHHHHHHANKKIEKQLQKDKQVYRATHRLLLLGAGESGKSTIVKQMRILHVNGGGDQDALRSRVLTSGIFETKFQVDKVNFHMFDVGGQRDARRKWIQCFNDVTAIIFVVASSSYNMVIREDNQTNRLQEALNLFKSIWNNRWLRTISVILFLNKQDLLAEKVLAGKSKIEDYFPEFARYTTPEDATPEPGEDPRVTRAKYFIRDEFLRISTASGDGRHYCYPHFTCAVDTENIRRVFNDCRDIIQRMHLRQYELL

SEQ ID NO: 12 - protein, 257 aa, synthetic construct
  REGION 1..257: note = MINI GS92
MGHHHHHHANKKIEKQLQKDKQVYRATHRLLLLGAGESGKSTIVKQMRILHVNGGGDQDALRSRVLTSGIFETKFQVDKVNFHMFDVGGQRDERRKWIQCFNDVTAIIFVVDSSSYNMVIREDNQTNRLQEALNLFKSIWNNRWLRTISVILFLNKQDLLAEKVLAGKSKIEDYFPEFARYTTPEDATPEPGEDPRVTRAKYFIRDEFLRISTASGDGRHYCYPHFTCAVDTENIRRVFNDCRDIIQRMHLRQYELL

SEQ ID NO: 13 - protein, 257 aa, synthetic construct
  REGION 1..257: note = MINI GS104
MGHHHHHHANKKIEKQLQKDKQVYRATHRLLLLGAGESGKSTIVKQMRILHVNGGGDQDALRSRVLTSGIFETKFQVDKVNFHMFDVGGQRDERRKWIQCFNDVTAIIFVVESSSYNMVIREDNQTNRLQEALNLFKSIWNNRWLRTISVILFLNKQDLLAEKVLAGKSKIEDYFPEFARYTTPEDATPEPGEDPRVTRAKYFIRDEFLRISTASGDGRHYCYPHFTCAVDTENIRRVFNDCRDIIQRMHLRQYELL

SEQ ID NO: 14 - protein, 257 aa, synthetic construct
  REGION 1..257: note = MINI GS117
MGHHHHHHANKKIEKQLQKDKQVYRATHRLLLLGAGESGKSTIVKQMRILHVNGGGDQDALRSRVLTSGIFETKFQVDKVNFHMFDVGGQRDERRKWIQCFNDVTAIIFVVASSDYNMVIREDNQTNRLQEALNLFKSIWNNRWLRTISVILFLNKQDLLAEKVLAGKSKIEDYFPEFARYTTPEDATPEPGEDPRVTRAKYFIRDEFLRISTASGDGRHYCYPHFTCAVDTENIRRVFNDCRDIIQRMHLRQYELL

SEQ ID NO: 15 - protein, 257 aa, synthetic construct
  REGION 1..257: note = MINI GS118
MGHHHHHHANKKIEKQLQKDKQVYRATHRLLLLGAGESGKSTIVKQMRILHVNGGGDQDALRSRVLTSGIFETKFQVDKVNFHMFDVGGQRDERRKWIQCFNDVTAIIFVVASSEYNMVIREDNQTNRLQEALNLFKSIWNNRWLRTISVILFLNKQDLLAEKVLAGKSKIEDYFPEFARYTTPEDATPEPGEDPRVTRAKYFIRDEFLRISTASGDGRHYCYPHFTCAVDTENIRRVFNDCRDIIQRMHLRQYELL

SEQ ID NO: 16 - protein, 247 aa, synthetic construct
  REGION 1..247: note = MINI GS105
MGHHHHHHANKKIEKQLQKDKQVYRATHRLLLLGAGESGKSTIVKQMRILHVNGGGDQDALRSRVLTSGIFETKFQVDKVNFHMFDVGGQRDERRKWIQCFNDVTAIIFVVASSSYNRLQEALNLFKSIWNNRWLRTISVILFLNKQDLLAEKVLAGKSKIEDYFPEFARYTTPEDATPEPGEDPRVTRAKYFIRDEFLRISTASGDGRHYCYPHFTCAVDTENIRRVFNDCRDIIQRMHLRQYELL

SEQ ID NO: 17 - protein, 257 aa, synthetic construct
  REGION 1..257: note = MINI GS94
MGHHHHHHANKKIEKQLQKDKQVYRATHRLLLLGAGESGKSTIVKQMRILHVNGGGDQDALRSRVLTSGIFETKFQVDKVNFHMFDVGGQRDERRKWIQCFNDVTAIIFVVASSSYNMVIREDNQTNRLQEALNDFKSIWNNRWLRTISVILFLNKQDLLAEKVLAGKSKIEDYFPEFARYTTPEDATPEPGEDPRVTRAKYFIRDEFLRISTASGDGRHYCYPHFTCAVDTENIRRVFNDCRDIIQRMHLRQYELL

SEQ ID NO: 18 - protein, 257 aa, synthetic construct
  REGION 1..257: note = MINI GS113
MGHHHHHHANKKIEKQLQKDKQVYRATHRLLLLGAGESGKSTIVKQMRILHVNGGGDQDALRSRVLTSGIFETKFQVDKVNFHMFDVGGQRDERRKWIQCFNDVTAIIFVVASSSYNMVIREDNQTNRLQEALNEFKSIWNNRWLRTISVILFLNKQDLLAEKVLAGKSKIEDYFPEFARYTTPEDATPEPGEDPRVTRAKYFIRDEFLRISTASGDGRHYCYPHFTCAVDTENIRRVFNDCRDIIQRMHLRQYELL

SEQ ID NO: 19 - protein, 242 aa, synthetic construct
  REGION 1..242: note = MINI GS161
MGHHHHHHANKKIEKQLQKDKQVYRATHRLLLLGAGESGKSTIVKQMRILHGGGGGETKFQVDKVNFHMFDVGGQRDERRKWIQCFNDVTAIIFVVASSSYNMVIREDNQTNRLQEALNLFKSIWNNRWLRTISVILFLNKQDLLAEKVLAGKSKIEDYFPEFARYTTPEDATPEPGEDPRVTRAKYFIRDEFLRISTASGDGRHYCYPHFTCAVDTENIRRVFNDCRDIIQRMHLRQYELL

SEQ ID NO: 20 - protein, 242 aa, synthetic construct
  REGION 1..242: note = MINI GS162
MGHHHHHHANKKIEKQLQKDKQVYRATHRLLLLGAGESGKSTIVKQMRILHGGGGGETKFQVDKVNFHMFDVGGQRDERRKWIQCFNDVTAIIFVVDSSSYNMVIREDNQTNRLQEALNLFKSIWNNRWLRTISVILFLNKQDLLAEKVLAGKSKIEDYFPEFARYTTPEDATPEPGEDPRVTRAKYFIRDEFLRISTASGDGRHYCYPHFTCAVDTENIRRVFNDCRDIIQRMHLRQYELL

SEQ ID NO: 21 - protein, 232 aa, synthetic construct
  REGION 1..232: note = MINI GS164
MGHHHHHHANKKIEKQLQKDKQVYRATHRLLLLGAGESGKSTIVKQMRILHGGGGGETKFQVDKVNFHMFDVGGQRDERRKWIQCFNDVTAIIFVVDSSSYNRLQEALNLFKSIWNNRWLRTISVILFLNKQDLLAEKVLAGKSKIEDYFPEFARYTTPEDATPEPGEDPRVTRAKYFIRDEFLRISTASGDGRHYCYPHFTCAVDTENIRRVFNDCRDIIQRMHLRQYELL

SEQ ID NO: 22 - protein, 232 aa, synthetic construct
  REGION 1..232: note = MINI GS165
MGHHHHHHANKKIEKQLQKDKQVYRATHRLLLLGAGESGKSTIVKQMRILHGGGGGETKFQVDKVNFHMFDVGGQRDERRKWIQCFNDVTAIIFVVDSSDYNRLQEALNLFKSIWNNRWLRTISVILFLNKQDLLAEKVLAGKSKIEDYFPEFARYTTPEDATPEPGEDPRVTRAKYFIRDEFLRISTASGDGRHYCYPHFTCAVDTENIRRVFNDCRDIIQRMHLRQYELL

SEQ ID NO: 23 - protein, 232 aa, synthetic construct
  REGION 1..232: note = MINI GS169
MGHHHHHHANKKIEKQLQKDKQVYRATHRLLLLGAGESGKSTIVKQMRILHGGGGGETKFQVDKVNFHMFDVGGQRDERRKWIQCFNDVTAIIFVVDSSDYNRLQEALNDFKSIWNNRWLRTISVILFLNKQDLLAEKVLAGKSKIEDYFPEFARYTTPEDATPEPGEDPRVTRAKYFIRDEFLRISTASGDGRHYCYPHFTCAVDTENIRRVFNDCRDIIQRMHLRQYELL

SEQ ID NO: 24 - protein, 232 aa, synthetic construct
  REGION 1..232: note = MINI GS183
MGHHHHHHANKKIEKQLQKDKQVYRATHRLLLLGADNSGKSTIVKQMRILHGGGGGETKFQVDKVNFHMFDVGGQRDERRKWIQCFNDVTAIIFVVDSSDYNRLQEALNDFKSIWNNRWLRTISVILFLNKQDLLAEKVLAGKSKIEDYFPEFARYTTPEDATPEPGEDPRVTRAKYFIRDEFLRISTASGDGRHYCYPHFTCAVDTENIRRVFNDCRDIIQRMHLRQYELL

SEQ ID NO: 25 - protein, 240 aa, synthetic construct
  REGION 1..240: note = MINI GS199
MGHHHHHHANKKIEKQLQKDKQVYRATHRLLLLGADNSGKSTIVKQMRILHGGGGGGGGTSGIFETKFQVDKVNFHMFDVGGQRDERRKWIQCFNDVTAIIFVVDSSDYNRLQEALNDFKSIWNNRWLRTISVILFLNKQDLLAEKVLAGKSKIEDYFPEFARYTTPEDATPEPGEDPRVTRAKYFIRDEFLRISTASGDGRHYCYPHFTCAVDTENIRRVFNDCRDIIQRMHLRQYELL

SEQ ID NO: 26 - protein, 240 aa, synthetic construct
  REGION 1..240: note = MINI GS254
MGHHHHHHANKKIEKQLQKDKQVYRATHRLLLLGADNSGKSTIVKQARILHGGGGGGGGTSGIFETKFQVDKVNFHMFDVGGQRDERRKWIQCFNDVTAIIFVVDSSDYNRLQEALNDFKSIWNNRWLRTISVILFLNKQDLLAEKVLAGKSKIEDYFPEFARYTTPEDATPEPGEDPRVTRAKYFIRDEFLRISTASGDGRHYCYPHFTCAVDTENIRRVFNDCRDIIQRMHLRQYELL

SEQ ID NO: 27 - protein, 240 aa, synthetic construct
  REGION 1..240: note = MINI GS350
MGHHHHHHANKKIEKQLQKDKQVYRATHRLLLLGADNSGKSTIVKQMRIYHGGGGGGGGTSGIFETKFQVDKVNFHMFDVGGQRDERRKWIQCFNDVTAIIFVVDSSDYNRLQEALNDFKSIWNNRWLRTISVILFLNKQDLLAEKVLAGKSKIEDYFPEFARYTTPEDATPEPGEDPRVTRAKYFIRDEFLRISTASGDGRHYCYPHFTCAVDTENIRRVFNDCRDIIQRMHLRQYELL

SEQ ID NO: 28 - protein, 240 aa, synthetic construct
  REGION 1..240: note = MINI GS340
MGHHHHHHANKKIEKQLQKDKQVYRATHRLLLLGADNSGKSTIVKQMRILHGGGGGGGGTSGIFETKFQVDKVNFHMFDVGGQRDERRKWIQCFNDVTAIIFVVDSSDYNRLQEALNDFKSIWNNRWLRTISVILFLNKQDLLAEKVLAGKSKIEDYFPEFARYTTPEDATPEPGEDPRVTRAKYFIRDEFLRISTASGDGRHYCYPHFTCAVDTENARRVFNDCRDIIQRMHLRQYELL

SEQ ID NO: 29 - protein, 240 aa, synthetic construct
  REGION 1..240: note = MINI GS303
MGHHHHHHANKKIEKQLQKDKQVYRATHRLLLLGADNSGKSTIVKQMRILHGGGGGGGGTSGIFETKFQVDKVNFHMFDVGGQRDERRKWIQCFNDVTAIIFVVDSSDYNRLQEALNDFKSIWNNRWLRTISVILFLNKQDLLAEKVLAGKSKIEDYFPEFARYTTPEDATPEPGEDPRVTRAKYFIRDEFLRISTASGDGRHYCYPHFTCAVDTENIRRIFNDCRDIIQRMHLRQYELL

SEQ ID NO: 30 - protein, 240 aa, synthetic construct
  REGION 1..240: note = MINI GS352
MGHHHHHHANKKIEKQLQKDKQVYRATHRLLLLGADNSGKSTIVKQMRIYHGGGGGGGGTSGIFETKFQVDKVNFHMFDVGGQRDERRKWIQCFNDVTAIIFVVDSSDYNRLQEALNDFKSIWNNRWLRTISVILFLNKQDLLAEKVLAGKSKIEDYFPEFARYTTPEDATPEPGEDPRVTRAKYFIRDEFLRISTASGDGRHYCYPHFTCAVDTENARRVFNDCRDIIQRMHLRQYELL

SEQ ID NO: 31 - protein, 240 aa, synthetic construct
  REGION 1..240: note = MINI GS345
MGHHHHHHANKKIEKQLQKDKQVYRATHRLLLLGADNSGKSTIVKQMRILHGGGGGGGGTSGIFETKFQVDKVNFHMFDVGGQRDERRKWIQCFNDVTAIIFVVDSSDYNRLQEALNDFKSIWNNRWLRTISVILFLNKQDLLAEKVLAGKSKIEDYFPEFARYTTPEDATPEPGEDPRVTRAKYFIRDEFLRISTASGDGRHYCYPHFTCAVDTENARRIFNDCRDIIQRMHLRQYELL

SEQ ID NO: 32 - protein, 243 aa, synthetic construct
  REGION 1..243: note = MINI GS389
MGHHHHHHENLYFQGIEKQLQKDKQVYRATHRLLLLGADNSGKSTIVKQARILHGGSGGSGGTSGIFETKFQVDKVNFHMFDVGGQRDERRKWIQCFNDVTAIIFVVDSSDYNRLQEALNDFKSIWNNRWLRTISVILFLNKQDLLAEKVLAGKSKIEDYFPEFARYTTPEDATPEPGEDPRVTRAKYFIRDEFLRISTASGDGRHYCYPHFTCAVDTENIRRIFNDCRDIIQRMHLRQYELL

SEQ ID NO: 33 - protein, 243 aa, synthetic construct
  REGION 1..243: note = MINI GS391
MGHHHHHHENLYFQGIEKQLQKDKQVYRATHRLLLLGADNSGKSTIVKQMRILHGGSGGSGGTSGIFETKFQVDKVNFHMFDVGGQRDERRKWIQCFNDVTAIIFVVDSSDYNRLQEALNDFKSIWNNRWLRTISVILFLNKQDLLAEKVLAGKSKIEDYFPEFARYTTPEDATPEPGEDPRVTRAKYFIRDEFLRISTASGDGRHYCYPHFTCAVDTENARRVFNDCRDIIQRMHLRQYELL

SEQ ID NO: 34 - protein, 243 aa, synthetic construct
  REGION 1..243: note = MINI GS393
MGHHHHHHENLYFQGIEKQLQKDKQVYRATHRLLLLGADNSGKSTIVKQMRILHGGSGGSGGTSGIFETKFQVDKVNFHMFDVGGQRDERRKWIQCFNDVTAIIFVVDSSDYNRLQEALNDFKSIWNNRWLRTISVILFLNKQDLLAEKVLAGKSKIEDYFPEFARYTTPEDATPEPGEDPRVTRAKYFIRDEFLRISTASGDGRHYCYPHFTCAVDTENARRIFNDCRDIIQRMHLRQYELL

SEQ ID NO: 35 - protein, 263 aa, synthetic construct
  REGION 1..263: note = MINI GS395
MGHHHHHHENLYFQGNSKTEDQRNEEKAQREANKKIEKQLQKDKQVYRATHRLLLLGADNSGKSTIVKQARILHGGSGGSGGTSGIFETKFQVDKVNFHMFDVGGQRDERRKWIQCFNDVTAIIFVVDSSDYNRLQEALNLFKSIWNNRWLRTISVILFLNKQDLLAEKVLAGKSKIEDYFPEFARYTTPEDATPEPGEDPRVTRAKYFIRDEFLRISTASGDGRHYCYPHFTCAVDTENIRRIFNDCRDIIQRMHLRQYELL

SEQ ID NO: 36 - protein, 263 aa, synthetic construct
  REGION 1..263: note = MINI GS397
MGHHHHHHENLYFQGNSKTEDQRNEEKAQREANKKIEKQLQKDKQVYRATHRLLLLGADNSGKSTIVKQMRILHGGSGGSGGTSGIFETKFQVDKVNFHMFDVGGQRDERRKWIQCFNDVTAIIFVVDSSDYNRLQEALNLFKSIWNNRWLRTISVILFLNKQDLLAEKVLAGKSKIEDYFPEFARYTTPEDATPEPGEDPRVTRAKYFIRDEFLRISTASGDGRHYCYPHFTCAVDTENARRVFNDCRDIIQRMHLRQYELL

SEQ ID NO: 37 - protein, 263 aa, synthetic construct
  REGION 1..263: note = MINI GS399
MGHHHHHHENLYFQGNSKTEDQRNEEKAQREANKKIEKQLQKDKQVYRATHRLLLLGADNSGKSTIVKQMRILHGGSGGSGGTSGIFETKFQVDKVNFHMFDVGGQRDERRKWIQCFNDVTAIIFVVDSSDYNRLQEALNLFKSIWNNRWLRTISVILFLNKQDLLAEKVLAGKSKIEDYFPEFARYTTPEDATPEPGEDPRVTRAKYFIRDEFLRISTASGDGRHYCYPHFTCAVDTENARRIFNDCRDIIQRMHLRQYELL

SEQ ID NO: 38 - protein, 243 aa, synthetic construct
  REGION 1..243: note = MINI GS404
MGHHHHHHENLYFQGIEKQLQKDKQVYRATHRLLLLGADNSGKSTIVKQMRILHGGSGGSGGTSGIFETKFQVDKVNFHMFDVGGQRDERRKWIQCFNDVTAIIFVVDSSDYNRLQEALNDFKSIWNNRWLRTISVILFLNKQDLLAEKVLAGKSKIEDYFPEFARYTTPEDATPEPGEDPRVTRAKYFIRDEFLRISTASGDGRHYCYPHFTCAVDTENIRRVFNDCRDIIQRMHLRQYELL

SEQ ID NO: 39 - protein, 263 aa, synthetic construct
  REGION 1..263: note = MINI GS406
MGHHHHHHENLYFQGNSKTEDQRNEEKAQREANKKIEKQLQKDKQVYRATHRLLLLGADNSGKSTIVKQMRILHGGSGGSGGTSGIFETKFQVDKVNFHMFDVGGQRDERRKWIQCFNDVTAIIFVVDSSDYNRLQEALNLFKSIWNNRWLRTISVILFLNKQDLLAEKVLAGKSKIEDYFPEFARYTTPEDATPEPGEDPRVTRAKYFIRDEFLRISTASGDGRHYCYPHFTCAVDTENIRRVFNDCRDIIQRMHLRQYELL

SEQ ID NO: 40 - protein, 243 aa, synthetic construct
  REGION 1..243: note = MINI GS410
MGHHHHHHENLYFQGIEKQLQKDKQVYRATHRLLLLGADNSGKSTIVKQMRIRHGGSGGSGGTSGIFETKFQVDKVNFHMFDVGGQRDERRKWIQCFNDVTAIIFVVDSSDYNRLQEALNDFKSIWNNRWLRTISVILFLNKQDLLAEKVLAGKSKIEDYFPEFARYTTPEDATPEPGEDPRVTRAKYFIRDEFLRISTASGDGRHYCYPHFTCAVDTENARRIFNDCRDIIQRMHLRQYELL

SEQ ID NO: 41 - protein, 243 aa, synthetic construct
  REGION 1..243: note = MINI GS414
MGHHHHHHENLYFQGIEKQLQKDKQVYRATHRLLLLGADNSGKSTIVKQMRIYHGGSGGSGGTSGIFETKFQVDKVNFHMFDVGGQRDERRKWIQCFNDVTAIIFVVDSSDYNRLQEALNDFKSIWNNRWLRTISVILFLNKQDLLAEKVLAGKSKIEDYFPEFARYTTPEDATPEPGEDPRVTRAKYFIRDEFLRISTASGDGRHYCYPHFTCAVDTENARRIFNDCRDIIQRMHLRQYELL

SEQ ID NO: 42 - protein, 263 aa, synthetic construct
  REGION 1..263: note = MINI GS418
MGHHHHHHENLYFQGNSKTEDQRNEEKAQREANKKIEKQLQKDKQVYRATHRLLLLGADNSGKSTIVKQMRIYHGGSGGSGGTSGIFETKFQVDKVNFHMFDVGGQRDERRKWIQCFNDVTAIIFVVDSSDYNRLQEALNLFKSIWNNRWLRTISVILFLNKQDLLAEKVLAGKSKIEDYFPEFARYTTPEDATPEPGEDPRVTRAKYFIRDEFLRISTASGDGRHYCYPHFTCAVDTENARRIFNDCRDIIQRMHLRQYELL

SEQ ID NO: 43 - protein, 230 aa, synthetic construct
  REGION 1..230: note = MINI GS431
MGHHHHHHENLYFQGATHRLLLLGADNSGKSTIVKQMRILHGGSGGSGGTSGIFETKFQVDKVNFHMFDVGGQRDERRKWIQCFNDVTAIIFVVDSSDYNRLQEALNDFKSIWNNRWLRTISVILFLNKQDLLAEKVLAGKSKIEDYFPEFARYTTPEDATPEPGEDPRVTRAKYFIRDEFLRISTASGDGRHYCYPHFTCAVDTENARRIFNDCRDIIQRMHLRQYELL

SEQ ID NO: 44 - protein, 236 aa, synthetic construct
  REGION 1..236: note = MINI GS432
MGHHHHHHENLYFQGIEKQLQKDKQVYRATHRLLLLGADNSGKSTIVKQMRILHGGGGGGETKFQVDKVNFHMFDVGGQRDERRKWIQCFNDVTAIIFVVDSSDYNRLQEALNDFKSIWNNRWLRTISVILFLNKQDLLAEKVLAGKSKIEDYFPEFARYTTPEDATPEPGEDPRVTRAKYFIRDEFLRISTASGDGRHYCYPHFTCAVDTENARRIFNDCRDIIQRMHLRQYELL

SEQ ID NO: 45 - protein, 223 aa, synthetic construct
  REGION 1..223: note = MINI GS433
MGHHHHHHENLYFQGATHRLLLLGADNSGKSTIVKQMRILHGGGGGGETKFQVDKVNFHMFDVGGQRDERRKWIQCFNDVTAIIFVVDSSDYNRLQEALNDFKSIWNNRWLRTISVILFLNKQDLLAEKVLAGKSKIEDYFPEFARYTTPEDATPEPGEDPRVTRAKYFIRDEFLRISTASGDGRHYCYPHFTCAVDTENARRIFNDCRDIIQRMHLRQYELL

SEQ ID NO: 46 - DNA, 867 bp, synthetic construct
  misc_feature 1..867: note = MINI GS55
  source 1..867: mol_type = other DNA
atgggtcaccaccatcatcaccatcatcaccaccatgaaaatctttatttccagtctggctgcctcgggaacagtaagaccgaggaccagcgcaacgaggagaaggcgcagcgtgaggccaacaaaaagatcgagaagcagctgcagaaggacaagcaggtctaccgggccacgcaccgcctgctgctgctgggtgctggagaatctggtaaaagcaccattgtgaagcagatgaggatcctgcatgttaatggcggaggtgatcaggacctgcttcgctgccgtgtcctgacttctggaatctttgagaccaagttccaggtcgacaaagtcaacttccacatgtttgacgtgggtggccagcgcgatgaacgccgcaagtggatccagtgcttcaacgatgtgactgccatcatcttcgtggtggccagcagcagctacaacatggtcatccgggaggacaaccagaccaaccgcctgcaggaggctctgaacctcttcaagagcatctggaacaacagatggctgcgcaccatctctgtgatcctgttcctcaacaagcaagatctgctcgctgagaaagtccttgctgggaaatcgaagattgaggactactttccagaatttgctcgctacactactcctgaggatgctactcccgagcccggagaggacccacgcgtgacccgggccaagtacttcattcgagatgagtttctgaggatcagcactgccagtggagatgggcgtcactactgctaccctcatttcacctgcgctgtggacactgagaacatccgccgtgtgttcaacgactgccgtgacatcattcagcgcatgcaccttcgtcagtacgagctgctctaa

SEQ ID NO: 47 - DNA, 774 bp, synthetic construct
  misc_feature 1..774: note = MINI GS77
  source 1..774: mol_type = other DNA
atgggtcaccaccatcatcaccatgccaacaaaaagatcgagaagcagctgcagaaggacaagcaggtctaccgggccacgcaccgcctgctgctgctgggtgctggagaatctggtaaaagcaccattgtgaagcagatgaggatcctgcatgttaatggcggaggtgatcaggacgcgcttcgctcccgtgtcctgacttctggaatctttgagaccaagttccaggtcgacaaagtcaacttccacatgtttgacgtgggtggccagcgcgatgaacgccgcaagtggatccagtgcttcaacgatgtgactgccatcatcttcgtggtggccagcagcagctacaacatggtcatccgggaggacaaccagaccaaccgcctgcaggaggctctgaacctcttcaagagcatctggaacaacagatggctgcgcaccatctctgtgatcctgttcctcaacaagcaagatctgctcgctgagaaagtccttgctgggaaatcgaagattgaggactactttccagaatttgctcgctacactactcctgaggatgctactcccgagcccggagaggacccacgcgtgacccgggccaagtacttcattcgagatgagtttctgaggatcagcactgccagtggagatgggcgtcactactgctaccctcatttcacctgcgctgtggacactgagaacatccgccgtgtgttcaacgactgccgtgacatcattcagcgcatgcaccttcgtcagtacgagctgctctaa

SEQ ID NO: 48 - DNA, 774 bp, synthetic construct
  misc_feature 1..774: note = MINI GS81
  source 1..774: mol_type = other DNA
atgggtcaccaccatcatcaccatgccaacaaaaagatcgagaagcagctgcagaaggacaagcaggtctaccgggccacgatccgcctgctgctgctgggtgctggagaatctggtaaaagcaccattgtgaagcagatgaggatcctgcatgttaatggcggaggtgatcaggacgcgcttcgctcccgtgtcctgacttctggaatctttgagaccaagttccaggtcgacaaagtcaacttccacatgtttgacgtgggtggccagcgcgatgaacgccgcaagtggatccagtgcttcaacgatgtgactgccatcatcttcgtggtggccagcagcagctacaacatggtcatccgggaggacaaccagaccaaccgcctgcaggaggctctgaacctcttcaagagcatctggaacaacagatggctgcgcaccatctctgtgatcctgttcctcaacaagcaagatctgctcgctgagaaagtccttgctgggaaatcgaagattgaggactactttccagaatttgctcgctacactactcctgaggatgctactcccgagcccggagaggacccacgcgtgacccgggccaagtacttcattcgagatgagtttctgaggatcagcactgccagtggagatgggcgtcactactgctaccctcatttcacctgcgctgtggacactgagaacatccgccgtgtgttcaacgactgccgtgacatcattcagcgcatgcaccttcgtcagtacgagctgctctaa

SEQ ID NO: 49 - DNA, 774 bp, synthetic construct
  misc_feature 1..774: note = MINI GS84
  source 1..774: mol_type = other DNA
atgggtcaccaccatcatcaccatgccaacaaaaagatcgagaagcagctgcagaaggacaagcaggtctaccgggccacggtccgcctgctgctgctgggtgctggagaatctggtaaaagcaccattgtgaagcagatgaggatcctgcatgttaatggcggaggtgatcaggacgcgcttcgctcccgtgtcctgacttctggaatctttgagaccaagttccaggtcgacaaagtcaacttccacatgtttgacgtgggtggccagcgcgatgaacgccgcaagtggatccagtgcttcaacgatgtgactgccatcatcttcgtggtggccagcagcagctacaacatggtcatccgggaggacaaccagaccaaccgcctgcaggaggctctgaacctcttcaagagcatctggaacaacagatggctgcgcaccatctctgtgatcctgttcctcaacaagcaagatctgctcgctgagaaagtccttgctgggaaatcgaagattgaggactactttccagaatttgctcgctacactactcctgaggatgctactcccgagcccggagaggacccacgcgtgacccgggccaagtacttcattcgagatgagtttctgaggatcagcactgccagtggagatgggcgtcactactgctaccctcatttcacctgcgctgtggacactgagaacatccgccgtgtgttcaacgactgccgtgacatcattcagcgcatgcaccttcgtcagtacgagctgctctaa

SEQ ID NO: 50 - DNA, 774 bp, synthetic construct
  misc_feature 1..774: note = MINI GS186
  source 1..774: mol_type = other DNA
atgggtcaccaccatcatcaccatgccaacaaaaagatcgagaagcagctgcagaaggacaagcaggtctaccgggccacgcaccgcctgctgctgctgggtcttggagaatctggtaaaagcaccattgtgaagcagatgaggatcctgcatgttaatggcggaggtgatcaggacgcgcttcgctcccgtgtcctgacttctggaatctttgagaccaagttccaggtcgacaaagtcaacttccacatgtttgacgtgggtggccagcgcgatgaacgccgcaagtggatccagtgcttcaacgatgtgactgccatcatcttcgtggtggccagcagcagctacaacatggtcatccgggaggacaaccagaccaaccgcctgcaggaggctctgaacctcttcaagagcatctggaacaacagatggctgcgcaccatctctgtgatcctgttcctcaacaagcaagatctgctcgctgagaaagtccttgctgggaaatcgaagattgaggactactttccagaatttgctcgctacactactcctgaggatgctactcccgagcccggagaggacccacgcgtgacccgggccaagtacttcattcgagatgagtttctgaggatcagcactgccagtggagatgggcgtcactactgctaccctcatttcacctgcgctgtggacactgagaacatccgccgtgtgttcaacgactgccgtgacatcattcagcgcatgcaccttcgtcagtacgagctgctctaa

SEQ ID NO: 51 - DNA, 774 bp, synthetic construct
  misc_feature 1..774: note = MINI GS130
  source 1..774: mol_type = other DNA
atgggtcaccaccatcatcaccatgccaacaaaaagatcgagaagcagctgcagaaggacaagcaggtctaccgggccacgcaccgcctgctgctgctgggtgctgatgaatctggtaaaagcaccattgtgaagcagatgaggatcctgcatgttaatggcggaggtgatcaggacgcgcttcgctcccgtgtcctgacttctggaatctttgagaccaagttccaggtcgacaaagtcaacttccacatgtttgacgtgggtggccagcgcgatgaacgccgcaagtggatccagtgcttcaacgatgtgactgccatcatcttcgtggtggccagcagcagctacaacatggtcatccgggaggacaaccagaccaaccgcctgcaggaggctctgaacctcttcaagagcatctggaacaacagatggctgcgcaccatctctgtgatcctgttcctcaacaagcaagatctgctcgctgagaaagtccttgctgggaaatcgaagattgaggactactttccagaatttgctcgctacactactcctgaggatgctactcccgagcccggagaggacccacgcgtgacccgggccaagtacttcattcgagatgagtttctgaggatcagcactgccagtggagatgggcgtcactactgctaccctcatttcacctgcgctgtggacactgagaacatccgccgtgtgttcaacgactgccgtgacatcattcagcgcatgcaccttcgtcagtacgagctgctctaa

SEQ ID NO: 52 - DNA, 774 bp, synthetic construct
  misc_feature 1..774: note = MINI GS116
  source 1..774: mol_type = other DNA
atgggtcaccaccatcatcaccatgccaacaaaaagatcgagaagcagctgcagaaggacaagcaggtctaccgggccacgcaccgcctgctgctgctgggtgctggaaattctggtaaaagcaccattgtgaagcagatgaggatcctgcatgttaatggcggaggtgatcaggacgcgcttcgctcccgtgtcctgacttctggaatctttgagaccaagttccaggtcgacaaagtcaacttccacatgtttgacgtgggtggccagcgcgatgaacgccgcaagtggatccagtgcttcaacgatgtgactgccatcatcttcgtggtggccagcagcagctacaacatggtcatccgggaggacaaccagaccaaccgcctgcaggaggctctgaacctcttcaagagcatctggaacaacagatggctgcgcaccatctctgtgatcctgttcctcaacaagcaagatctgctcgctgagaaagtccttgctgggaaatcgaagattgaggactactttccagaatttgctcgctacactactcctgaggatgctactcccgagcccggagaggacccacgcgtgacccgggccaagtacttcattcgagatgagtttctgaggatcagcactgccagtggagatgggcgtcactactgctaccctcatttcacctgcgctgtggacactgagaacatccgccgtgtgttcaacgactgccgtgacatcattcagcgcatgcaccttcgtcagtacgagctgctctaa

SEQ ID NO: 53 - DNA, 774 bp, synthetic construct
  misc_feature 1..774: note = MINI GS134
  source 1..774: mol_type = other DNA
atgggtcaccaccatcatcaccatgccaacaaaaagatcgagaagcagctgcagaaggacaagcaggtctaccgggccacgcaccgcctgctgctgctgggtgctggagaatctggtaaaagcaccattgtgaagcagatgaggatcctgcatgttaatggcggaggtgatcaggacgcgcttcgctccgctgtcctgacttctggaatctttgagaccaagttccaggtcgacaaagtcaacttccacatgtttgacgtgggtggccagcgcgatgaacgccgcaagtggatccagtgcttcaacgatgtgactgccatcatcttcgtggtggccagcagcagctacaacatggtcatccgggaggacaaccagaccaaccgcctgcaggaggctctgaacctcttcaagagcatctggaacaacagatggctgcgcaccatctctgtgatcctgttcctcaacaagcaagatctgctcgctgagaaagtccttgctgggaaatcgaagattgaggactactttccagaatttgctcgctacactactcctgaggatgctactcccgagcccggagaggacccacgcgtgacccgggccaagtacttcattcgagatgagtttctgaggatcagcactgccagtggagatgggcgtcactactgctaccctcatttcacctgcgctgtggacactgagaacatccgccgtgtgttcaacgactgccgtgacatcattcagcgcatgcaccttcgtcagtacgagctgctctaa

SEQ ID NO: 54 - DNA, 774 bp, synthetic construct
  misc_feature 1..774: note = MINI GS111
  source 1..774: mol_type = other DNA
atgggtcaccaccatcatcaccatgccaacaaaaagatcgagaagcagctgcagaaggacaagcaggtctaccgggccacgcaccgcctgctgctgctgggtgctggagaatctggtaaaagcaccattgtgaagcagatgaggatcctgcatgttaatggcggaggtgatcaggacgcgcttcgctcccgtgtcctgacttctggaatctttgagaccaagttccaggtcgacaaagtcaacttccacatgtttgacgtgggtgcccagcgcgatgaacgccgcaagtggatccagtgcttcaacgatgtgactgccatcatcttcgtggtggccagcagcagctacaacatggtcatccgggaggacaaccagaccaaccgcctgcaggaggctctgaacctcttcaagagcatctggaacaacagatggctgcgcaccatctctgtgatcctgttcctcaacaagcaagatctgctcgctgagaaagtccttgctgggaaatcgaagattgaggactactttccagaatttgctcgctacactactcctgaggatgctactcccgagcccggagaggacccacgcgtgacccgggccaagtacttcattcgagatgagtttctgaggatcagcactgccagtggagatgggcgtcactactgctaccctcatttcacctgcgctgtggacactgagaacatccgccgtgtgttcaacgactgccgtgacatcattcagcgcatgcaccttcgtcagtacgagctgctctaa

SEQ ID NO: 55 - DNA, 768 bp, synthetic construct
  misc_feature 1..768: note = MINI GS98
  source 1..768: mol_type = other DNA
atgggtcaccaccatcatcaccatgccaacaaaaagatcgagaagcagctgcagaaggacaagcaggtctaccgggccacgcaccgcctgctgctgctgggtgctggagaatctggtaaaagcaccattgtgaagcagatgaggatcctgcatgttaatggcggaggtgatcaggacgcgcttcgctcccgtgtcctgacttctggaatctttgagaccaagttccaggtcgacaaagtcaacttccacatgtttgacgtgggtggcggagggcgccgcaagtggatccagtgcttcaacgatgtgactgccatcatcttcgtggtggccagcagcagctacaacatggtcatccgggaggacaaccagaccaaccgcctgcaggaggctctgaacctcttcaagagcatctggaacaacagatggctgcgcaccatctctgtgatcctgttcctcaacaagcaagatctgctcgctgagaaagtccttgctgggaaatcgaagattgaggactactttccagaatttgctcgctacactactcctgaggatgctactcccgagcccggagaggacccacgcgtgacccgggccaagtacttcattcgagatgagtttctgaggatcagcactgccagtggagatgggcgtcactactgctaccctcatttcacctgcgctgtggacactgagaacatccgccgtgtgttcaacgactgccgtgacatcattcagcgcatgcaccttcgtcagtacgagctgctctaa

SEQ ID NO: 56 - DNA, 774 bp, synthetic construct
  misc_feature 1..774: note = MINI GS175
  source 1..774: mol_type = other DNA
atgggtcaccaccatcatcaccatgccaacaaaaagatcgagaagcagctgcagaaggacaagcaggtctaccgggccacgcaccgcctgctgctgctgggtgctggagaatctggtaaaagcaccattgtgaagcagatgaggatcctgcatgttaatggcggaggtgatcaggacgcgcttcgctcccgtgtcctgacttctggaatctttgagaccaagttccaggtcgacaaagtcaacttccacatgtttgacgtgggtggccagcgcgatgcacgccgcaagtggatccagtgcttcaacgatgtgactgccatcatcttcgtggtggccagcagcagctacaacatggtcatccgggaggacaaccagaccaaccgcctgcaggaggctctgaacctcttcaagagcatctggaacaacagatggctgcgcaccatctctgtgatcctgttcctcaacaagcaagatctgctcgctgagaaagtccttgctgggaaatcgaagattgaggactactttccagaatttgctcgctacactactcctgaggatgctactcccgagcccggagaggacccacgcgtgacccgggccaagtacttcattcgagatgagtttctgaggatcagcactgccagtggagatgggcgtcactactgctaccctcatttcacctgcgctgtggacactgagaacatccgccgtgtgttcaacgactgccgtgacatcattcagcgcatgcaccttcgtcagtacgagctgctctaa

SEQ ID NO: 57 - DNA, 774 bp, synthetic construct
  misc_feature 1..774: note = MINI GS92
  source 1..774: mol_type = other DNA
atgggtcaccaccatcatcaccatgccaacaaaaagatcgagaagcagctgcagaaggacaagcaggtctaccgggccacgcaccgcctgctgctgctgggtgctggagaatctggtaaaagcaccattgtgaagcagatgaggatcctgcatgttaatggcggaggtgatcaggacgcgcttcgctcccgtgtcctgacttctggaatctttgagaccaagttccaggtcgacaaagtcaacttccacatgtttgacgtgggtggccagcgcgatgaacgccgcaagtggatccagtgcttcaacgatgtgactgccatcatcttcgtggtggacagcagcagctacaacatggtcatccgggaggacaaccagaccaaccgcctgcaggaggctctgaacctcttcaagagcatctggaacaacagatggctgcgcaccatctctgtgatcctgttcctcaacaagcaagatctgctcgctgagaaagtccttgctgggaaatcgaagattgaggactactttccagaatttgctcgctacactactcctgaggatgctactcccgagcccggagaggacccacgcgtgacccgggccaagtacttcattcgagatgagtttctgaggatcagcactgccagtggagatgggcgtcactactgctaccctcatttcacctgcgctgtggacactgagaacatccgccgtgtgttcaacgactgccgtgacatcattcagcgcatgcaccttcgtcagtacgagctgctctaa

SEQ ID NO: 58 - DNA, 774 bp, synthetic construct
  misc_feature 1..774: note = MINI GS104
  source 1..774: mol_type = other DNA
atgggtcaccaccatcatcaccatgccaacaaaaagatcgagaagcagctgcagaaggacaagcaggtctaccgggccacgcaccgcctgctgctgctgggtgctggagaatctggtaaaagcaccattgtgaagcagatgaggatcctgcatgttaatggcggaggtgatcaggacgcgcttcgctcccgtgtcctgacttctggaatctttgagaccaagttccaggtcgacaaagtcaacttccacatgtttgacgtgggtggccagcgcgatgaacgccgcaagtggatccagtgcttcaacgatgtgactgccatcatcttcgtggtggagagcagcagctacaacatggtcatccgggaggacaaccagaccaaccgcctgcaggaggctctgaacctcttcaagagcatctggaacaacagatggctgcgcaccatctctgtgatcctgttcctcaacaagcaagatctgctcgctgagaaagtccttgctgggaaatcgaagattgaggactactttccagaatttgctcgctacactactcctgaggatgctactcccgagcccggagaggacccacgcgtgacccgggccaagtacttcattcgagatgagtttctgaggatcagcactgccagtggagatgggcgtcactactgctaccctcatttcacctgcgctgtggacactgagaacatccgccgtgtgttcaacgactgccgtgacatcattcagcgcatgcaccttcgtcagtacgagctgctctaa

SEQ ID NO: 59 - DNA, 774 bp, synthetic construct
  misc_feature 1..774: note = MINI GS117
  source 1..774: mol_type = other DNA
atgggtcaccaccatcatcaccatgccaacaaaaagatcgagaagcagctgcagaaggacaagcaggtctaccgggccacgcaccgcctgctgctgctgggtgctggagaatctggtaaaagcaccattgtgaagcagatgaggatcctgcatgttaatggcggaggtgatcaggacgcgcttcgctcccgtgtcctgacttctggaatctttgagaccaagttccaggtcgacaaagtcaacttccacatgtttgacgtgggtggccagcgcgatgaacgccgcaagtggatccagtgcttcaacgatgtgactgccatcatcttcgtggtggccagcagcgactacaacatggtcatccgggaggacaaccagaccaaccgcctgcaggaggctctgaacctcttcaagagcatctggaacaacagatggctgcgcaccatctctgtgatcctgttcctcaacaagcaagatctgctcgctgagaaagtccttgctgggaaatcgaagattgaggactactttccagaatttgctcgctacactactcctgaggatgctactcccgagcccggagaggacccacgcgtgacccgggccaagtacttcattcgagatgagtttctgaggatcagcactgccagtggagatgggcgtcactactgctaccctcatttcacctgcgctgtggacactgagaacatccgccgtgtgttcaacgactgccgtgacatcattcagcgcatgcaccttcgtcagtacgagctgctctaa

SEQ ID NO: 60 - DNA, 774 bp, synthetic construct
  misc_feature 1..774: note = MINI GS118
  source 1..774: mol_type = other DNA
atgggtcaccaccatcatcaccatgccaacaaaaagatcgagaagcagctgcagaaggacaagcaggtctaccgggccacgcaccgcctgctgctgctgggtgctggagaatctggtaaaagcaccattgtgaagcagatgaggatcctgcatgttaatggcggaggtgatcaggacgcgcttcgctcccgtgtcctgacttctggaatctttgagaccaagttccaggtcgacaaagtcaacttccacatgtttgacgtgggtggccagcgcgatgaacgccgcaagtggatccagtgcttcaacgatgtgactgccatcatcttcgtggtggccagcagcgagtacaacatggtcatccgggaggacaaccagaccaaccgcctgcaggaggctctgaacctcttcaagagcatctggaacaacagatggctgcgcaccatctctgtgatcctgttcctcaacaagcaagatctgctcgctgagaaagtccttgctgggaaatcgaagattgaggactactttccagaatttgctcgctacactactcctgaggatgctactcccgagcccggagaggacccacgcgtgacccgggccaagtacttcattcgagatgagtttctgaggatcagcactgccagtggagatgggcgtcactactgctaccctcatttcacctgcgctgtggacactgagaacatccgccgtgtgttcaacgactgccgtgacatcattcagcgcatgcaccttcgtcagtacgagctgctctaa

SEQ ID NO: 61 - DNA, 744 bp, synthetic construct
  misc_feature 1..744: note = MINI GS105
  source 1..744: mol_type = other DNA
atgggtcaccaccatcatcaccatgccaacaaaaagatcgagaagcagctgcagaaggacaagcaggtctaccgggccacgcaccgcctgctgctgctgggtgctggagaatctggtaaaagcaccattgtgaagcagatgaggatcctgcatgttaatggcggaggtgatcaggacgcgcttcgctcccgtgtcctgacttctggaatctttgagaccaagttccaggtcgacaaagtcaacttccacatgtttgacgtgggtggccagcgcgatgaacgccgcaagtggatccagtgcttcaacgatgtgactgccatcatcttcgtggtggccagcagcagctacaaccgcctgcaggaggctctgaacctcttcaagagcatctggaacaacagatggctgcgcaccatctctgtgatcctgttcctcaacaagcaagatctgctcgctgagaaagtccttgctgggaaatcgaagattgaggactactttccagaatttgctcgctacactactcctgaggatgctactcccgagcccggagaggacccacgcgtgacccgggccaagtacttcattcgagatgagtttctgaggatcagcactgccagtggagatgggcgtcactactgctaccctcatttcacctgcgctgtggacactgagaacatccgccgtgtgttcaacgactgccgtgacatcattcagcgcatgcaccttcgtcagtacgagctgctctaa

SEQ ID NO: 62 - DNA, 774 bp, synthetic construct
  misc_feature 1..774: note = MINI GS94
  source 1..774: mol_type = other DNA
atgggtcaccaccatcatcaccatgccaacaaaaagatcgagaagcagctgcagaaggacaagcaggtctaccgggccacgcaccgcctgctgctgctgggtgctggagaatctggtaaaagcaccattgtgaagcagatgaggatcctgcatgttaatggcggaggtgatcaggacgcgcttcgctcccgtgtcctgacttctggaatctttgagaccaagttccaggtcgacaaagtcaacttccacatgtttgacgtgggtggccagcgcgatgaacgccgcaagtggatccagtgcttcaacgatgtgactgccatcatcttcgtggtggccagcagcagctacaacatggtcatccgggaggacaaccagaccaaccgcctgcaggaggctctgaacgacttcaagagcatctggaacaacagatggctgcgcaccatctctgtgatcctgttcctcaacaagcaagatctgctcgctgagaaagtccttgctgggaaatcgaagattgaggactactttccagaatttgctcgctacactactcctgaggatgctactcccgagcccggagaggacccacgcgtgacccgggccaagtacttcattcgagatgagtttctgaggatcagcactgccagtggagatgggcgtcactactgctaccctcatttcacctgcgctgtggacactgagaacatccgccgtgtgttcaacgactgccgtgacatcattcagcgcatgcaccttcgtcagtacgagctgctctaa

SEQ ID NO: 63 - DNA, 774 bp, synthetic construct
  misc_feature 1..774: note = MINI GS113
  source 1..774: mol_type = other DNA
atgggtcaccaccatcatcaccatgccaacaaaaagatcgagaagcagctgcagaaggacaagcaggtctaccgggccacgcaccgcctgctgctgctgggtgctggagaatctggtaaaagcaccattgtgaagcagatgaggatcctgcatgttaatggcggaggtgatcaggacgcgcttcgctcccgtgtcctgacttctggaatctttgagaccaagttccaggtcgacaaagtcaacttccacatgtttgacgtgggtggccagcgcgatgaacgccgcaagtggatccagtgcttcaacgatgtgactgccatcatcttcgtggtggccagcagcagctacaacatggtcatccgggaggacaaccagaccaaccgcctgcaggaggctctgaacgagttcaagagcatctggaacaacagatggctgcgcaccatctctgtgatcctgttcctcaacaagcaagatctgctcgctgagaaagtccttgctgggaaatcgaagattgaggactactttccagaatttgctcgctacactactcctgaggatgctactcccgagcccggagaggacccacgcgtgacccgggccaagtacttcattcgagatgagtttctgaggatcagcactgccagtggagatgggcgtcactactgctaccctcatttcacctgcgctgtggacactgagaacatccgccgtgtgttcaacgactgccgtgacatcattcagcgcatgcaccttcgtcagtacgagctgctctaa

SEQ ID NO: 64 - DNA, 729 bp, synthetic construct
  misc_feature 1..729: note = MINI GS161
  source 1..729: mol_type = other DNA
atgggtcaccaccatcatcaccatgccaacaaaaagatcgagaagcagctgcagaaggacaagcaggtctaccgggccacgcaccgcctgctgctgctgggtgctggagaatctggtaaaagcaccattgtgaagcagatgaggatcctgcatgggggaggtggaggcgagaccaagttccaggtggacaaagtcaacttccacatgtttgacgtgggtggccagcgcgatgaacgccgcaagtggatccagtgcttcaacgatgtgactgccatcatcttcgtggtggccagcagcagctacaacatggtcatccgggaggacaaccagaccaaccgcctgcaggaggctctgaacctcttcaagagcatctggaacaacagatggctgcgcaccatctctgtgatcctgttcctcaacaagcaagatctgctcgctgagaaagtccttgctgggaaatcgaagattgaggactactttccagaatttgctcgctacactactcctgaggatgctactcccgagcccggagaggacccacgcgtgacccgggccaagtacttcattcgagatgagtttctgaggatcagcactgccagtggagatgggcgtcactactgctaccctcatttcacctgcgctgtggacactgagaacatccgccgtgtgttcaacgactgccgtgacatcattcagcgcatgcaccttcgtcagtacgagctgctctaa

SEQ ID NO: 65 - DNA, 729 bp, synthetic construct
  misc_feature 1..729: note = MINI GS162
  source 1..729: mol_type = other DNA
atgggtcaccaccatcatcaccatgccaacaaaaagatcgagaagcagctgcagaaggacaagcaggtctaccgggccacgcaccgcctgctgctgctgggtgctggagaatctggtaaaagcaccattgtgaagcagatgaggatcctgcatgggggaggtggaggcgagaccaagttccaggtggacaaagtcaacttccacatgtttgacgtgggtggccagcgcgatgaacgccgcaagtggatccagtgcttcaacgatgtgactgccatcatcttcgtggtggacagcagcagctacaacatggtcatccgggaggacaaccagaccaaccgcctgcaggaggctctgaacctcttcaagagcatctggaacaacagatggctgcgcaccatctctgtgatcctgttcctcaacaagcaagatctgctcgctgagaaagtccttgctgggaaatcgaagattgaggactactttccagaatttgctcgctacactactcctgaggatgctactcccgagcccggagaggacccacgcgtgacccgggccaagtacttcattcgagatgagtttctgaggatcagcactgccagtggagatgggcgtcactactgctaccctcatttcacctgcgctgtggacactgagaacatccgccgtgtgttcaacgactgccgtgacatcattcagcgcatgcaccttcgtcagtacgagctgctctaa

SEQ ID NO: 66 - DNA, 699 bp, synthetic construct
  misc_feature 1..699: note = MINI GS164
  source 1..699: mol_type = other DNA
atgggtcaccaccatcatcaccatgccaacaaaaagatcgagaagcagctgcagaaggacaagcaggtctaccgggccacgcaccgcctgctgctgctgggtgctggagaatctggtaaaagcaccattgtgaagcagatgaggatcctgcatgggggaggtggaggcgagaccaagttccaggtggacaaagtcaacttccacatgtttgacgtgggtggccagcgcgatgaacgccgcaagtggatccagtgcttcaacgatgtgactgccatcatcttcgtggtggacagcagcagctacaaccgcctgcaggaggctctgaacctcttcaagagcatctggaacaacagatggctgcgcaccatctctgtgatcctgttcctcaacaagcaagatctgctcgctgagaaagtccttgctgggaaatcgaagattgaggactactttccagaatttgctcgctacactactcctgaggatgctactcccgagcccggagaggacccacgcgtgacccgggccaagtacttcattcgagatgagtttctgaggatcagcactgccagtggagatgggcgtcactactgctaccctcatttcacctgcgctgtggacactgagaacatccgccgtgtgttcaacgactgccgtgacatcattcagcgcatgcaccttcgtcagtacgagctgctctaa

SEQ ID NO: 67 - DNA, 699 bp, synthetic construct
  misc_feature 1..699: note = MINI GS165
  source 1..699: mol_type = other DNA
atgggtcaccaccatcatcaccatgccaacaaaaagatcgagaagcagctgcagaaggacaagcaggtctaccgggccacgcaccgcctgctgctgctgggtgctggagaatctggtaaaagcaccattgtgaagcagatgaggatcctgcatgggggaggtggaggcgagaccaagttccaggtggacaaagtcaacttccacatgtttgacgtgggtggccagcgcgatgaacgccgcaagtggatccagtgcttcaacgatgtgactgccatcatcttcgtggtggacagcagcgattacaaccgcctgcaggaggctctgaacctcttcaagagcatctggaacaacagatggctgcgcaccatctctgtgatcctgttcctcaacaagcaagatctgctcgctgagaaagtccttgctgggaaatcgaagattgaggactactttccagaatttgctcgctacactactcctgaggatgctactcccgagcccggagaggacccacgcgtgacccgggccaagtacttcattcgagatgagtttctgaggatcagcactgccagtggagatgggcgtcactactgctaccctcatttcacctgcgctgtggacactgagaacatccgccgtgtgttcaacgactgccgtgacatcattcagcgcatgcaccttcgtcagtacgagctgctctaa

SEQ ID NO: 68 - DNA, 699 bp, synthetic construct
  misc_feature 1..699: note = MINI GS169
  source 1..699: mol_type = other DNA
atgggtcaccaccatcatcaccatgccaacaaaaagatcgagaagcagctgcagaaggacaagcaggtctaccgggccacgcaccgcctgctgctgctgggtgctggagaatctggtaaaagcaccattgtgaagcagatgaggatcctgcatgggggaggtggaggcgagaccaagttccaggtggacaaagtcaacttccacatgtttgacgtgggtggccagcgcgatgaacgccgcaagtggatccagtgcttcaacgatgtgactgccatcatcttcgtggtggacagcagcgattacaaccgcctgcaggaggctctgaacgacttcaagagcatctggaacaacagatggctgcgcaccatctctgtgatcctgttcctcaacaagcaagatctgctcgctgagaaagtccttgctgggaaatcgaagattgaggactactttccagaatttgctcgctacactactcctgaggatgctactcccgagcccggagaggacccacgcgtgacccgggccaagtacttcattcgagatgagtttctgaggatcagcactgccagtggagatgggcgtcactactgctaccctcatttcacctgcgctgtggacactgagaacatccgccgtgtgttcaacgactgccgtgacatcattcagcgcatgcaccttcgtcagtacgagctgctctaa

SEQ ID NO: 69 - DNA, 699 bp, synthetic construct
  misc_feature 1..699: note = MINI GS183
  source 1..699: mol_type = other DNA
atgggtcaccaccatcatcaccatgccaacaaaaagatcgagaagcagctgcagaaggacaagcaggtctaccgggccacgcaccgcctgctgctgctgggtgctgataattctggtaaaagcaccattgtgaagcagatgaggatcctgcatgggggaggtggaggcgagaccaagttccaggtggacaaagtcaacttccacatgtttgacgtgggtggccagcgcgatgaacgccgcaagtggatccagtgcttcaacgatgtgactgccatcatcttcgtggtggacagcagcgattacaaccgcctgcaggaggctctgaacgacttcaagagcatctggaacaacagatggctgcgcaccatctctgtgatcctgttcctcaacaagcaagatctgctcgctgagaaagtccttgctgggaaatcgaagattgaggactactttccagaatttgctcgctacactactcctgaggatgctactcccgagcccggagaggacccacgcgtgacccgggccaagtacttcattcgagatgagtttctgaggatcagcactgccagtggagatgggcgtcactactgctaccctcatttcacctgcgctgtggacactgagaacatccgccgtgtgttcaacgactgccgtgacatcattcagcgcatgcaccttcgtcagtacgagctgctctaa

SEQ ID NO: 70 - DNA, 723 bp, synthetic construct
  misc_feature 1..723: note = MINI GS199
  source 1..723: mol_type = other DNA
atgggtcaccaccatcatcaccatgccaacaaaaagatcgagaagcagctgcagaaggacaagcaggtctaccgggccacgcaccgcctgctgctgctgggtgctgataattctggtaaaagcaccattgtgaagcagatgaggatcctgcatggtgggggaggcgggggcggaggtacttctggaatctttgagaccaagttccaggtggacaaagtcaacttccacatgtttgacgtgggtggccagcgcgatgaacgccgcaagtggatccagtgcttcaacgatgtgactgccatcatcttcgtggtggacagcagcgattacaaccgcctgcaggaggctctgaacgacttcaagagcatctggaacaacagatggctgcgcaccatctctgtgatcctgttcctcaacaagcaagatctgctcgctgagaaagtccttgctgggaaatcgaagattgaggactactttccagaatttgctcgctacactactcctgaggatgctactcccgagcccggagaggacccacgcgtgacccgggccaagtacttcattcgagatgagtttctgaggatcagcactgccagtggagatgggcgtcactactgctaccctcatttcacctgcgctgtggacactgagaacatccgccgtgtgttcaacgactgccgtgacatcattcagcgcatgcaccttcgtcagtacgagctgctctaa

SEQ ID NO: 71 - DNA, 723 bp, synthetic construct
  misc_feature 1..723: note = MINI GS254
  source 1..723: mol_type = other DNA
atgggtcaccaccatcatcaccatgccaacaaaaagatcgagaagcagctgcagaaggacaagcaggtctaccgggccacgcaccgcctgctgctgctgggtgctgataattctggtaaaagcaccattgtgaagcaggcgaggatcctgcatggtgggggaggcgggggcggaggtacttctggaatctttgagaccaagttccaggtggacaaagtcaacttccacatgtttgacgtgggtggccagcgcgatgaacgccgcaagtggatccagtgcttcaacgatgtgactgccatcatcttcgtggtggacagcagcgattacaaccgcctgcaggaggctctgaacgacttcaagagcatctggaacaacagatggctgcgcaccatctctgtgatcctgttcctcaacaagcaagatctgctcgctgagaaagtccttgctgggaaatcgaagattgaggactactttccagaatttgctcgctacactactcctgaggatgctactcccgagcccggagaggacccacgcgtgacccgggccaagtacttcattcgagatgagtttctgaggatcagcactgccagtggagatgggcgtcactactgctaccctcatttcacctgcgctgtggacactgagaacatccgccgtgtgttcaacgactgccgtgacatcattcagcgcatgcaccttcgtcagtacgagctgctctaa

SEQ ID NO: 72 - DNA, 723 bp, synthetic construct
  misc_feature 1..723: note = MINI GS350
  source 1..723: mol_type = other DNA
atgggtcaccaccatcatcaccatgccaacaaaaagatcgagaagcagctgcagaaggacaagcaggtctaccgggccacgcaccgcctgctgctgctgggtgctgataattctggtaaaagcaccattgtgaagcagatgaggatctaccatggtgggggaggcgggggcggaggtacttctggaatctttgagaccaagttccaggtggacaaagtcaacttccacatgtttgacgtgggtggccagcgcgatgaacgccgcaagtggatccagtgcttcaacgatgtgactgccatcatcttcgtggtggacagcagcgattacaaccgcctgcaggaggctctgaacgacttcaagagcatctggaacaacagatggctgcgcaccatctctgtgatcctgttcctcaacaagcaagatctgctcgctgagaaagtccttgctgggaaatcgaagattgaggactactttccagaatttgctcgctacactactcctgaggatgctactcccgagcccggagaggacccacgcgtgacccgggccaagtacttcattcgagatgagtttctgaggatcagcactgccagtggagatgggcgtcactactgctaccctcatttcacctgcgctgtggacactgagaacatccgccgtgtgttcaacgactgccgtgacatcattcagcgcatgcaccttcgtcagtacgagctgctctaa

SEQ ID NO: 73 - DNA, 723 bp, synthetic construct
  misc_feature 1..723: note = MINI GS340
  source 1..723: mol_type = other DNA
atgggtcaccaccatcatcaccatgccaacaaaaagatcgagaagcagctgcagaaggacaagcaggtctaccgggccacgcaccgcctgctgctgctgggtgctgataattctggtaaaagcaccattgtgaagcagatgaggatcctgcatggtgggggaggcgggggcggaggtacttctggaatctttgagaccaagttccaggtggacaaagtcaacttccacatgtttgacgtgggtggccagcgcgatgaacgccgcaagtggatccagtgcttcaacgatgtgactgccatcatcttcgtggtggacagcagcgattacaaccgcctgcaggaggctctgaacgacttcaagagcatctggaacaacagatggctgcgcaccatctctgtgatcctgttcctcaacaagcaagatctgctcgctgagaaagtccttgctgggaaatcgaagattgaggactactttccagaatttgctcgctacactactcctgaggatgctactcccgagcccggagaggacccacgcgtgacccgggccaagtacttcattcgagatgagtttctgaggatcagcactgccagtggagatgggcgtcactactgctaccctcatttcacctgcgctgtggacactgagaacgcccgccgtgtgttcaacgactgccgtgacatcattcagcgcatgcaccttcgtcagtacgagctgctctaa

SEQ ID NO: 74 - DNA, 723 bp, synthetic construct; identical to SEQ ID NO: 73
  misc_feature 1..723: note = MINI GS303
  source 1..723: mol_type = other DNA

SEQ ID NO: 75 - DNA, 723 bp, synthetic construct
  misc_feature 1..723: note = MINI GS352
  source 1..723: mol_type = other DNA
atgggtcaccaccatcatcaccatgccaacaaaaagatcgagaagcagctgcagaaggacaagcaggtctaccgggccacgcaccgcctgctgctgctgggtgctgataattctggtaaaagcaccattgtgaagcagatgaggatctaccatggtgggggaggcgggggcggaggtacttctggaatctttgagaccaagttccaggtggacaaagtcaacttccacatgtttgacgtgggtggccagcgcgatgaacgccgcaagtggatccagtgcttcaacgatgtgactgccatcatcttcgtggtggacagcagcgattacaaccgcctgcaggaggctctgaacgacttcaagagcatctggaacaacagatggctgcgcaccatctctgtgatcctgttcctcaacaagcaagatctgctcgctgagaaagtccttgctgggaaatcgaagattgaggactactttccagaatttgctcgctacactactcctgaggatgctactcccgagcccggagaggacccacgcgtgacccgggccaagtacttcattcgagatgagtttctgaggatcagcactgccagtggagatgggcgtcactactgctaccctcatttcacctgcgctgtggacactgagaacgcccgccgtgtgttcaacgactgccgtgacatcattcagcgcatgcaccttcgtcagtacgagctgctctaa

SEQ ID NO: 76 - DNA, 723 bp, synthetic construct
  misc_feature 1..723: note = MINI GS345
  source 1..723: mol_type = other DNA
atgggtcaccaccatcatcaccatgccaacaaaaagatcgagaagcagctgcagaaggacaagcaggtctaccgggccacgcaccgcctgctgctgctgggtgctgataattctggtaaaagcaccattgtgaagcagatgaggatcctgcatggtgggggaggcgggggcggaggtacttctggaatctttgagaccaagttccaggtggacaaagtcaacttccacatgtttgacgtgggtggccagcgcgatgaacgccgcaagtggatccagtgcttcaacgatgtgactgccatcatcttcgtggtggacagcagcgattacaaccgcctgcaggaggctctgaacgacttcaagagcatctggaacaacagatggctgcgcaccatctctgtgatcctgttcctcaacaagcaagatctgctcgctgagaaagtccttgctgggaaatcgaagattgaggactactttccagaatttgctcgctacactactcctgaggatgctactcccgagcccggagaggacccacgcgtgacccgggccaagtacttcattcgagatgagtttctgaggatcagcactgccagtggagatgggcgtcactactgctaccctcatttcacctgcgctgtggacactgagaacgcccgccgtatcttcaacgactgccgtgacatcattcagcgcatgcaccttcgtcagtacgagctgctctaa

SEQ ID NO: 77 - DNA, 732 bp, synthetic construct
  misc_feature 1..732: note = MINI GS389
  source 1..732: mol_type = other DNA
atgggtcaccaccatcatcaccatgaaaatctttatttccagggtatcgagaagcagctgcagaaggacaagcaggtctaccgggccacgcaccgcctgctgctgctgggtgctgataattctggtaaaagcaccattgtgaagcaggcgaggatcctgcatggtgggagtggcgggagcggaggtacttctggaatctttgagaccaagttccaggtggacaaagtcaacttccacatgtttgacgtgggtggccagcgcgatgaacgccgcaagtggatccagtgcttcaacgatgtgactgccatcatcttcgtggtggacagcagcgattacaaccgcctgcaggaggctctgaacgacttcaagagcatctggaacaacagatggctgcgcaccatctctgtgatcctgttcctcaacaagcaagatctgctcgctgagaaagtccttgctgggaaatcgaagattgaggactactttccagaatttgctcgctacactactcctgaggatgctactcccgagcccggagaggacccacgcgtgacccgggccaagtacttcattcgagatgagtttctgaggatcagcactgccagtggagatgggcgtcactactgctaccctcatttcacctgcgctgtggacactgagaacatccgccgtatcttcaacgactgccgtgacatcattcagcgcatgcaccttcgtcagtacgagctgctctaa

SEQ ID NO: 78 - DNA, 732 bp, synthetic construct
  misc_feature 1..732: note = MINI GS391
  source 1..732: mol_type = other DNA
atgggtcaccaccatcatcaccatgaaaatctttatttccagggtatcgagaagcagctgcagaaggacaagcaggtctaccgggccacgcaccgcctgctgctgctgggtgctgataattctggtaaaagcaccattgtgaagcagatgaggatcctgcatggtgggagtggcgggagcggaggtacttctggaatctttgagaccaagttccaggtggacaaagtcaacttccacatgtttgacgtgggtggccagcgcgatgaacgccgcaagtggatccagtgcttcaacgatgtgactgccatcatcttcgtggtggacagcagcgattacaaccgcctgcaggaggctctgaacgacttcaagagcatctggaacaacagatggctgcgcaccatctctgtgatcctgttcctcaacaagcaagatctgctcgctgagaaagtccttgctgggaaatcgaagattgaggactactttccagaatttgctcgctacactactcctgaggatgctactcccgagcccggagaggacccacgcgtgacccgggccaagtacttcattcgagatgagtttctgaggatcagcactgccagtggagatgggcgtcactactgctaccctcatttcacctgcgctgtggacactgagaacgcccgccgtgtgttcaacgactgccgtgacatcattcagcgcatgcaccttcgtcagtacgagctgctctaa

SEQ ID NO: 79 - DNA, 732 bp, synthetic construct
  misc_feature 1..732: note = MINI GS393
  source 1..732: mol_type = other DNA
atgggtcaccaccatcatcaccatgaaaatctttatttccagggtatcgagaagcagctgcagaaggacaagcaggtctaccgggccacgcaccgcctgctgctgctgggtgctgataattctggtaaaagcaccattgtgaagcagatgaggatcctgcatggtgggagtggcgggagcggaggtacttctggaatctttgagaccaagttccaggtggacaaagtcaacttccacatgtttgacgtgggtggccagcgcgatgaacgccgcaagtggatccagtgcttcaacgatgtgactgccatcatcttcgtggtggacagcagcgattacaaccgcctgcaggaggctctgaacgacttcaagagcatctggaacaacagatggctgcgcaccatctctgtgatcctgttcctcaacaagcaagatctgctcgctgagaaagtccttgctgggaaatcgaagattgaggactactttccagaatttgctcgctacactactcctgaggatgctactcccgagcccggagaggacccacgcgtgacccgggccaagtacttcattcgagatgagtttctgaggatcagcactgccagtggagatgggcgtcactactgctaccctcatttcacctgcgctgtggacactgagaacgcccgccgtatcttcaacgactgccgtgacatcattcagcgcatgcaccttcgtcagtacgagctgctctaa

SEQ ID NO: 80 - DNA, 792 bp, synthetic construct
  misc_feature 1..792: note = MINI GS395
  source 1..792: mol_type = other DNA
atgggtcaccaccatcatcaccatgaaaatctttatttccagggtaacagtaagaccgaggaccagcgcaacgaggagaaggcgcagcgtgaggccaacaaaaagatcgagaagcagctgcagaaggacaagcaggtctaccgggccacgcaccgcctgctgctgctgggtgctgataattctggtaaaagcaccattgtgaagcaggcgaggatcctgcatggtgggagtggcgggagcggaggtacttctggaatctttgagaccaagttccaggtggacaaagtcaacttccacatgtttgacgtgggtggccagcgcgatgaacgccgcaagtggatccagtgcttcaacgatgtgactgccatcatcttcgtggtggacagcagcgattacaaccgcctgcaggaggctctgaacctcttcaagagcatctggaacaacagatggctgcgcaccatctctgtgatcctgttcctcaacaagcaagatctgctcgctgagaaagtccttgctgggaaatcgaagattgaggactactttccagaatttgctcgctacactactcctgaggatgctactcccgagcccggagaggacccacgcgtgacccgggccaagtacttcattcgagatgagtttctgaggatcagcactgccagtggagatgggcgtcactactgctaccctcatttcacctgcgctgtggacactgagaacatccgccgtatcttcaacgactgccgtgacatcattcagcgcatgcaccttcgtcagtacgagctgctctaa

SEQ ID NO: 81 - DNA, 792 bp, synthetic construct
  misc_feature 1..792: note = MINI GS397
  source 1..792: mol_type = other DNA
atgggtcaccaccatcatcaccatgaaaatctttatttccagggtaacagtaagaccgaggaccagcgcaacgaggagaaggcgcagcgtgaggccaacaaaaagatcgagaagcagctgcagaaggacaagcaggtctaccgggccacgcaccgcctgctgctgctgggtgctgataattctggtaaaagcaccattgtgaagcagatgaggatcctgcatggtgggagtggcgggagcggaggtacttctggaatctttgagaccaagttccaggtggacaaagtcaacttccacatgtttgacgtgggtggccagcgcgatgaacgccgcaagtggatccagtgcttcaacgatgtgactgccatcatcttcgtggtggacagcagcgattacaaccgcctgcaggaggctctgaacctcttcaagagcatctggaacaacagatggctgcgcaccatctctgtgatcctgttcctcaacaagcaagatctgctcgctgagaaagtccttgctgggaaatcgaagattgaggactactttccagaatttgctcgctacactactcctgaggatgctactcccgagcccggagaggacccacgcgtgacccgggccaagtacttcattcgagatgagtttctgaggatcagcactgccagtggagatgggcgtcactactgctaccctcatttcacctgcgctgtggacactgagaacgcccgccgtgtgttcaacgactgccgtgacatcattcagcgcatgcaccttcgtcagtacgagctgctctaa

SEQ ID NO: 82 - DNA, 792 bp, synthetic construct
  misc_feature 1..792: note = MINI GS399
  source 1..792: mol_type = other DNA
atgggtcaccaccatcatcaccatgaaaatctttatttccagggtaacagtaagaccgaggaccagcgcaacgaggagaaggcgcagcgtgaggccaacaaaaagatcgagaagcagctgcagaaggacaagcaggtctaccgggccacgcaccgcctgctgctgctgggtgctgataattctggtaaaagcaccattgtgaagcagatgaggatcctgcatggtgggagtggcgggagcggaggtacttctggaatctttgagaccaagttccaggtggacaaagtcaacttccacatgtttgacgtgggtggccagcgcgatgaacgccgcaagtggatccagtgcttcaacgatgtgactgccatcatcttcgtggtggacagcagcgattacaaccgcctgcaggaggctctgaacctcttcaagagcatctggaacaacagatggctgcgcaccatctctgtgatcctgttcctcaacaagcaagatctgctcgctgagaaagtccttgctgggaaatcgaagattgaggactactttccagaatttgctcgctacactactcctgaggatgctactcccgagcccggagaggacccacgcgtgacccgggccaagtacttcattcgagatgagtttctgaggatcagcactgccagtggagatgggcgtcactactgctaccctcatttcacctgcgctgtggacactgagaacgcccgccgtatcttcaacgactgccgtgacatcattcagcgcatgcaccttcgtcagtacgagctgctctaa

SEQ ID NO: 83 - DNA, 732 bp, synthetic construct
  misc_feature 1..732: note = MINI GS404
  source 1..732: mol_type = other DNA
atgggtcaccaccatcatcaccatgaaaatctttatttccagggtatcgagaagcagctgcagaaggacaagcaggtctaccgggccacgcaccgcctgctgctgctgggtgctgataattctggtaaaagcaccattgtgaagcagatgaggatcctgcatggtgggagtggcgggagcggaggtacttctggaatctttgagaccaagttccaggtggacaaagtcaacttccacatgtttgacgtgggtggccagcgcgatgaacgccgcaagtggatccagtgcttcaacgatgtgactgccatcatcttcgtggtggacagcagcgattacaaccgcctgcaggaggctctgaacgacttcaagagcatctggaacaacagatggctgcgcaccatctctgtgatcctgttcctcaacaagcaagatctgctcgctgagaaagtccttgctgggaaatcgaagattgaggactactttccagaatttgctcgctacactactcctgaggatgctactcccgagcccggagaggacccacgcgtgacccgggccaagtacttcattcgagatgagtttctgaggatcagcactgccagtggagatgggcgtcactactgctaccctcatttcacctgcgctgtggacactgagaacatccgccgtgtgttcaacgactgccgtgacatcattcagcgcatgcaccttcgtcagtacgagctgctctaa

SEQ ID NO: 84 - DNA, 792 bp, synthetic construct
  misc_feature 1..792: note = MINI GS406
  source 1..792: mol_type = other DNA
atgggtcaccaccatcatcaccatgaaaatctttatttccagggtaacagtaagaccgaggaccagcgcaacgaggagaaggcgcagcgtgaggccaacaaaaagatcgagaagcagctgcagaaggacaagcaggtctaccgggccacgcaccgcctgctgctgctgggtgctgataattctggtaaaagcaccattgtgaagcagatgaggatcctgcatggtgggagtggcgggagcggaggtacttctggaatctttgagaccaagttccaggtggacaaagtcaacttccacatgtttgacgtgggtggccagcgcgatgaacgccgcaagtggatccagtgcttcaacgatgtgactgccatcatcttcgtggtggacagcagcgattacaaccgcctgcaggaggctctgaacctcttcaagagcatctggaacaacagatggctgcgcaccatctctgtgatcctgttcctcaacaagcaagatctgctcgctgagaaagtccttgctgggaaatcgaagattgaggactactttccagaatttgctcgctacactactcctgaggatgctactcccgagcccggagaggacccacgcgtgacccgggccaagtacttcattcgagatgagtttctgaggatcagcactgccagtggagatgggcgtcactactgctaccctcatttcacctgcgctgtggacactgagaacatccgccgtgtgttcaacgactgccgtgacatcattcagcgcatgcaccttcgtcagtacgagctgctctaa

SEQ ID NO: 85 - DNA, 732 bp, synthetic construct
  misc_feature 1..732: note = MINI GS410
  source 1..732: mol_type = other DNA
atgggtcaccaccatcatcaccatgaaaatctttatttccagggtatcgagaagcagctgcagaaggacaagcaggtctaccgggccacgcaccgcctgctgctgctgggtgctgataattctggtaaaagcaccattgtgaagcagatgaggatccggcatggtgggagtggcgggagcggaggtacttctggaatctttgagaccaagttccaggtggacaaagtcaacttccacatgtttgacgtgggtggccagcgcgatgaacgccgcaagtggatccagtgcttcaacgatgtgactgccatcatcttcgtggtggacagcagcgattacaaccgcctgcaggaggctctgaacgacttcaagagcatctggaacaacagatggctgcgcaccatctctgtgatcctgttcctcaacaagcaagatctgctcgctgagaaagtccttgctgggaaatcgaagattgaggactactttccagaatttgctcgctacactactcctgaggatgctactcccgagcccggagaggacccacgcgtgacccgggccaagtacttcattcgagatgagtttctgaggatcagcactgccagtggagatgggcgtcactactgctaccctcatttcacctgcgctgtggacactgagaacgcccgccgtatcttcaacgactgccgtgacatcattcagcgcatgcaccttcgtcagtacgagctgctctaa

SEQ ID NO: 86 - DNA, 732 bp, synthetic construct
  misc_feature 1..732: note = MINI GS414
  source 1..732: mol_type = other DNA
atgggtcaccaccatcatcaccatgaaaatctttatttccagggtatcgagaagcagctgcagaaggacaagcaggtctaccgggccacgcaccgcctgctgctgctgggtgctgataattctggtaaaagcaccattgtgaagcagatgaggatctaccatggtgggagtggcgggagcggaggtacttctggaatctttgagaccaagttccaggtggacaaagtcaacttccacatgtttgacgtgggtggccagcgcgatgaacgccgcaagtggatccagtgcttcaacgatgtgactgccatcatcttcgtggtggacagcagcgattacaaccgcctgcaggaggctctgaacgacttcaagagcatctggaacaacagatggctgcgcaccatctctgtgatcctgttcctcaacaagcaagatctgctcgctgagaaagtccttgctgggaaatcgaagattgaggactactttccagaatttgctcgctacactactcctgaggatgctactcccgagcccggagaggacccacgcgtgacccgggccaagtacttcattcgagatgagtttctgaggatcagcactgccagtggagatgggcgtcactactgctaccctcatttcacctgcgctgtggacactgagaacgcccgccgtatcttcaacgactgccgtgacatcattcagcgcatgcaccttcgtcagtacgagctgctctaa

SEQ ID NO: 87 - DNA, 792 bp, synthetic construct
  misc_feature 1..792: note = MINI GS418
  source 1..792: mol_type = other DNA
atgggtcaccaccatcatcaccatgaaaatctttatttccagggtaacagtaagaccgaggaccagcgcaacgaggagaaggcgcagcgtgaggccaacaaaaagatcgagaagcagctgcagaaggacaagcaggtctaccgggccacgcaccgcctgctgctgctgggtgctgataattctggtaaaagcaccattgtgaagcagatgaggatctaccatggtgggagtggcgggagcggaggtacttctggaatctttgagaccaagttccaggtggacaaagtcaacttccacatgtttgacgtgggtggccagcgcgatgaacgccgcaagtggatccagtgcttcaacgatgtgactgccatcatcttcgtggtggacagcagcgattacaaccgcctgcaggaggctctgaacctcttcaagagcatctggaacaacagatggctgcgcaccatctctgtgatcctgttcctcaacaagcaagatctgctcgctgagaaagtccttgctgggaaatcgaagattgaggactactttccagaatttgctcgctacactactcctgaggatgctactcccgagcccggagaggacccacgcgtgacccgggccaagtacttcattcgagatgagtttctgaggatcagcactgccagtggagatgggcgtcactactgctaccctcatttcacctgcgctgtggacactgagaacgcccgccgtatcttcaacgactgccgtgacatcattcagcgcatgcaccttcgtcagtacgagctgctctaa

SEQ ID NO: 88 - DNA, 693 bp, synthetic construct
  misc_feature 1..693: note = MINI GS431
  source 1..693: mol_type = other DNA
atgggtcaccaccatcatcaccatgaaaatctttatttccagggtgccacgcaccgcctgctgctgctgggtgctgataattctggtaaaagcaccattgtgaagcagatgaggatcctgcatggtgggagtggcgggagcggaggtacttctggaatctttgagaccaagttccaggtggacaaagtcaacttccacatgtttgacgtgggtggccagcgcgatgaacgccgcaagtggatccagtgcttcaacgatgtgactgccatcatcttcgtggtggacagcagcgattacaaccgcctgcaggaggctctgaacgacttcaagagcatctggaacaacagatggctgcgcaccatctctgtgatcctgttcctcaacaagcaagatctgctcgctgagaaagtccttgctgggaaatcgaagattgaggactactttccagaatttgctcgctacactactcctgaggatgctactcccgagcccggagaggacccacgcgtgacccgggccaagtacttcattcgagatgagtttctgaggatcagcactgccagtggagatgggcgtcactactgctaccctcatttcacctgcgctgtggacactgagaacgcccgccgtatcttcaacgactgccgtgacatcattcagcgcatgcaccttcgtcagtacgagctgctctaa

SEQ ID NO: 89 - DNA, 711 bp, synthetic construct
  misc_feature 1..711: note = MINI GS432
  source 1..711: mol_type = other DNA
atgggtcaccaccatcatcaccatgaaaatctttatttccagggtatcgagaagcagctgcagaaggacaagcaggtctaccgggccacgcaccgcctgctgctgctgggtgctgataattctggtaaaagcaccattgtgaagcagatgaggatcctgcatggtgggggtggcgggggcgagaccaagttccaggtggacaaagtcaacttccacatgtttgacgtgggtggccagcgcgatgaacgccgcaagtggatccagtgcttcaacgatgtgactgccatcatcttcgtggtggacagcagcgattacaaccgcctgcaggaggctctgaacgacttcaagagcatctggaacaacagatggctgcgcaccatctctgtgatcctgttcctcaacaagcaagatctgctcgctgagaaagtccttgctgggaaatcgaagattgaggactactttccagaatttgctcgctacactactcctgaggatgctactcccgagcccggagaggacccacgcgtgacccgggccaagtacttcattcgagatgagtttctgaggatcagcactgccagtggagatgggcgtcactactgctaccctcatttcacctgcgctgtggacactgagaacgcccgccgtatcttcaacgactgccgtgacatcattcagcgcatgcaccttcgtcagtacgagctgctctaa

SEQ ID NO: 90 - DNA, 672 bp, synthetic construct
  misc_feature 1..672: note = MINI GS433
  source 1..672: mol_type = other DNA
atgggtcaccaccatcatcaccatgaaaatctttatttccagggtgccacgcaccgcctgctgctgctgggtgctgataattctggtaaaagcaccattgtgaagcagatgaggatcctgcatggtgggggtggcgggggcgagaccaagttccaggtggacaaagtcaacttccacatgtttgacgtgggtggccagcgcgatgaacgccgcaagtggatccagtgcttcaacgatgtgactgccatcatcttcgtggtggacagcagcgattacaaccgcctgcaggaggctctgaacgacttcaagagcatctggaacaacagatggctgcgcaccatctctgtgatcctgttcctcaacaagcaagatctgctcgctgagaaagtccttgctgggaaatcgaagattgaggactactttccagaatttgctcgctacactactcctgaggatgctactcccgagcccggagaggacccacgcgtgacccgggccaagtacttcattcgagatgagtttctgaggatcagcactgccagtggagatgggcgtcactactgctaccctcatttcacctgcgctgtggacactgagaacgcccgccgtatcttcaacgactgccgtgacatcattcagcgcatgcaccttcgtcagtacgagctgctctaa

SEQ ID NO: 91 - protein, 229 aa, synthetic construct
  REGION 1..229: note = Mini Gs v2
MIEKQLQKDKQVYRATHRLLLLGADNSGKSTIVKQMRILHGGSGGSGGTSGIFETKFQVDKVNFHMFDVGGQRDERRKWIQCFNDVTAIIFVVDSSDYNRLQEALNDFKSIWNNRWLRTISVILFLNKQDLLAEKVLAGKSKIEDYFPEFARYTTPEDATPEPGEDPRVTRAKYFIRDEFLRISTASGDGRHYCYPHFTCAVDTENARRIFNDCRDIIQRMHLRQYELL

SEQ ID NO: 92 - protein, 394 aa, Homo sapiens
  REGION 1..394: note = Human G alpha s
MGCLGNSKTEDQRNEEKAQREANKKIEKQLQKDKQVYRATHRLLLLGAGESGKSTIVKQMRILHVNGFNGEGGEEDPQAARSNSDGEKATKVQDIKNNLKEAIETIVAAMSNLVPPVELANPENQFRVDYILSVMNVPDFDFPPEFYEHAKALWEDEGVRACYERSNEYQLIDCAQYFLDKIDVIKQADYVPSDQDLLRCRVLTSGIFETKFQVDKVNFHMFDVGGQRDERRKWIQCFNDVTAIIFVVASSSYNMVIREDNQTNRLQEALNLFKSIWNNRWLRTISVILFLNKQDLLAEKVLAGKSKIEDYFPEFARYTTPEDATPEPGEDPRVTRAKYFIRDEFLRISTASGDGRHYCYPHFTCAVDTENIRRVFNDCRDIIQRMHLRQYELL

SEQ ID NO: 93 - protein, 8 aa, synthetic construct
  REGION 1..8: note = Linker
GGSGGSGG

SEQ ID NO: 94 - protein, 8 aa, synthetic construct
  REGION 1..8: note = Linker
GGGGGGGG

SEQ ID NO: 95 - protein, 263 aa, Homo sapiens
  REGION 1..263: note = s
MGCLGNSKTEDQRNEEKAQREANKKIEKQLQKDKQVYRATHRLLLLGAGESGKSTIVKQMRILHGGSGGSGGTSGIFETKFQVDKVNFHMFDVGGQRDERRKWIQCFNDVTAIIFVVASSSYNMVIREDNQTNRLQEALNLFKSIWNNRWLRTISVILFLNKQDLLAEKVLAGKSKIEDYFPEFARYTTPEDATPEPGEDPRVTRAKYFIRDEFLRISTASGDGRHYCYPHFTCAVDTENIRRVFNDCRDIIQRMHLRQYELL

SEQ ID NO: 96 - protein, 265 aa, Homo sapiens
  REGION 1..265: note = olf
MGCLGGNSKTTEDQGVDEKERREANKKIEKQLQKERLAYKATHRLLLLGAGESGKSTIVKQMRILHGGSGGSGGTSGIFETRFQVDKVNFHMFDVGGQRDERRKWIQCFNDVTAIIYVAACSSYNMVIREDNNTNRLRESLDLFESIWNNRWLRTISIILFLNKQDMLAEKVLAGKSKIEDYFPEYANYTVPEDATPDAGEDPKVTRAKFFIRDLFLRISTATGDGKHYCYPHFTCAVDTENIRRVFNDCRDIIQRMHLKQYELL

SEQ ID NO: 97 - protein, 239 aa, Homo sapiens
  REGION 1..239: note = i1
MGCTLSAEDKAAVERSKMIDRNLREDGEKAAREVKLLLLGAGESGKSTIVKQMKIIHGGGGGGGGTTGIVETHFTFKDLHFKMFDVGGQRSERKKWIHCFEGVAAIIFCVALSDYDLVLAEDEEMNRMHESMKLFDSICNNKWFTDTSIILFLNKKDLFEEKIKKSPLTICYPEYAGSNTYEEAAAYIQCQFEDLNKRKDTKEIYTHFTCATDTKNVQFVFDAVTDVIIKNNLKDCGLF

SEQ ID NO: 98 - protein, 238 aa, Homo sapiens
  REGION 1..238: note = o1
MGCTLSAEERAALERSKAIEKNLKEDGISAAKDVKLLLLGAGESGKSTIVKQMKIIHGGSGGSGGTTGIVETHFTFKNLHFRLFDVGGQRSERKKWIHCFEDVTAIIFCVALSGYDQVLHEDETTNRMHESLMLFDSICNNKFFIDTSIILFLNKKDLFGEKIKKSPLTICFPEYTGPNTYEDAAAYIQAQFESKNRSPNKEIYCHMTCATDTNNIQVVFDAVTDIIIANNLRGCGLY

SEQ ID NO: 99 - protein, 235 aa, Homo sapiens
  REGION 1..235: note = t1
MGAGASAEEKHSRELEKKLKEDAEKDARTVKLLLLGAGESGKSTIVKQMKIIHGGSGGSGGTTGIIETQFSFKDLNFRMFDVGGQRSERKKWIHCFEGVTCIIFIAALSAYDMVLVEDDEVNRMHESLHLFNSICNHRYFATTSIVLFLNKKDVFFEKIKKAHLSICFPDYDGPNTYEDAGNYIKVQFLELNMRRDVKEIYSHMTCATDTQNVKFVFDAVTDIIIKENLKDCGLF

SEQ ID NO: 100 - protein, 239 aa, Homo sapiens
  REGION 1..239: note = z
MGCRQSSEEKEAARRSRRIDRHLRSESQRQRREIKLLLLGTSNSGKSTIVKQMKIIHGGGGGGGGTTGIVENKFTFKELTFKMVDVGGQRSERKKWIHCFEGVTAIIFCVELSGYDLKLYEDNQTSRMAESLRLFDSICNNNWFINTSLILFLNKKDLLAEKIRRIPLTICFPEYKGQNTYEEAAVYIQRQFEDLNRNKETKEIYSHFTCATDTSNIQFVFDAVTDVIIQNNLKYIGLC

SEQ ID NO: 101 - protein, 263 aa, Homo sapiens
  REGION 1..263: note = 12
MSGVVRTLSRCLLPAEAGGARERRAGSGARDAEREARRRSRDIDALLARERRAVRRLVKILLLGAGESGKSTFLKQMRIIHGGSGGSGGTKGIVEHDFVIKKIPFKMVDVGGQRSQRQKWFQCFDGITSILFMVSSSEYDQVLMEDRRTNRLVESMNIFETIVNNKLFFNVSIILFLNKMDLLVEKVKTVSIKKHFPDFRGDPHRLEDVQRYLVQCFDRKRRNRSKPLFHHFTTAIDTENVRFVFHAVKDTILQENLKDIMLQ

SEQ ID NO: 102 - protein, 245 aa, Homo sapiens
  REGION 1..245: note = q
MTLESIMACCLSEEAKEARRINDEIERQLRRDKRDARRELKLLLLGTGESGKSTFIKQMRIIHGGGGGGGGTTGIIEYPFDLQSVIFRMVDVGGQRSERRKWIHCFENVTSIMFLVALSEYDQVLVESDNENRMEESKALFRTIITYPWFQNSSVILFLNKKDLLEEKIMYSHLVDYFPEYDGPQRDAQAAREFILKMFVDLNPDSDKIIYSHFTCATDTENIRFVFAAVKDTILQLNLKEYNLV

SEQ ID NO: 103 - protein, 260 aa, Homo sapiens
  REGION 1..260: note = 16
MARSLTWRCCPWCLTEDEKAAARVDQEINRILLEQKKQDRGELKLLLLGPGESGKSTFIKQMRIIHGGGGGGGGTTGINEYCFSVQKTNLRIVDVGGQKSERKKWIHCFENVIALIYLASLSEYDQCLEENNQENRMKESLALFGTILELPWFKSTSVILFLNKTDILEEKIPTSHLATYFPSFQGPKQDAEAAKRFILDMYTRMYTGCVDGPEGSKKGARSRRLFSHYTCATDTQNIRKVFKDVRDSVLARYLDEINLL

SEQ ID NO: 104 - protein, 243 aa, synthetic construct; identical to SEQ ID NO: 34
  REGION 1..243: note = Mini-Gs393

SEQ ID NO: 105 - protein, 243 aa, synthetic construct
  REGION 1..243: note = Mini-Golf6
MGHHHHHHENLYFQGIEKQLQKERLAYKATHRLLLLGADNSGKSTIVKQMRILHGGSGGSGGTSGIFETRFQVDKVNFHMFDVGGQRDERRKWIQCFNDVTAIIYVADCSDYNRLRESLDDFESIWNNRWLRTISIILFLNKQDMLAEKVLAGKSKIEDYFPEYANYTVPEDATPDAGEDPKVTRAKFFIRDLFLRISTATGDGKHYCYPHFTCAVDTENARRIFNDCRDIIQRMHLKQYELL

SEQ ID NO: 106 - protein, 243 aa, synthetic construct
  REGION 1..243: note = Mini-Gs/q57
MGHHHHHHENLYFQGIEKQLQKDKQVYRATHRLLLLGADNSGKSTIVKQMRILHGGSGGSGGTSGIFETKFQVDKVNFHMFDVGGQRDERRKWIQCFNDVTAIIFVVDSSDYNRLQEALNDFKSIWNNRWLRTISVILFLNKQDLLAEKVLAGKSKIEDYFPEFARYTTPEDATPEPGEDPRVTRAKYFIRDEFLRISTASGDGRHYCYPHFTCAVDTENARRIFNDCRDIIQRMHLREYNLV

SEQ ID NO: 107 - protein, 243 aa, synthetic construct
  REGION 1..243: note = Mini-Gs/q58
MGHHHHHHENLYFQGIEKQLQKDKQVYRATHRLLLLGADNSGKSTIVKQMRILHGGSGGSGGTSGIFETKFQVDKVNFHMFDVGGQRDERRKWIQCFNDVTAIIFVVDSSDYNRLQEALNDFKSIWNNRWLRTISVILFLNKQDLLAEKVLAGKSKIEDYFPEFARYTTPEDATPEPGEDPRVTRAKYFIRDEFLRISTASGDGRHYCYPHFTCAVDTENARRIFAAVKDTILQLNLKEYNLV

SEQ ID NO: 108 - protein, 243 aa, synthetic construct
  REGION 1..243: note = Mini-Gs/q70
MGHHHHHHENLYFQGIEKQLQKDKQVYRATHRLLLLGADNSGKSTIVKQMRILHGGSGGSGGTSGIFETKFQVDKVNFHMFDVGGQRDERRKWIQCFNDVTAIIFVVDSSDYNRLQEALNDFKSIWNNRWLRTISVILFLNKQDLLAEKVLAGKSKIEDYFPEFARYTTPEDATPEPGEDPRVTRAKYFIRDEFLRISTASGDGRHYCYPHFTCAVDTENARRIFNDCKDIILQMNLREYNLV

SEQ ID NO: 109 - protein, 243 aa, synthetic construct
  REGION 1..243: note = Mini-Gs/q71
MGHHHHHHENLYFQGIEKQLQKDKQVYRRTLRLLLLGADNSGKSTIVKQMRILHGGSGGSGGTSGIFETKFQVDKVNFHMFDVGGQRDERRKWIQCFNDVTAIIFVVDSSDYNRLQEALNDFKSIWNNRWLRTISVILFLNKQDLLAEKVLAGKSKIEDYFPEFARYTTPEDATPEPGEDPRVTRAKYFIRKEFVDISTASGDGRHICYPHFTCAVDTENARRIFNDCKDIILQMNLREYNLV

SEQ ID NO: 110 - protein, 241 aa, synthetic construct
  REGION 1..241: note = Mini-Gi146
MGHHHHHHENLYFQGTLSAEDKAAVERSKMIDRNLREDGEKAAREVKLLLLGADNSGKSTIVKQMKIIHGGGGGGGGTTGIVETHFTFKDLHFKMFDVGGQRSERKKWIHCFEDVAAIIFCVDLSDYNRMHESMKLFDSICNNKWFTDTSIILFLNKKDLFEEKIKKSPLTICYQEYAGSNTYEEAAAYIQCQFEDLNKRKDTKEIYTHFTCATDTKNAQFIFDAVTDVIIKNNLKDCGLF

SEQ ID NO: 111 - protein, 243 aa, synthetic construct
  REGION 1..243: note = Mini-Gs/i143
MGHHHHHHENLYFQGIEKQLQKDKQVYRATHRLLLLGADNSGKSTIVKQMRILHGGSGGSGGTSGIFETKFQVDKVNFHMFDVGGQRDERRKWIQCFNDVTAIIFVVDSSDYNRLQEALNDFKSIWNNRWLRTISVILFLNKQDLLAEKVLAGKSKIEDYFPEFARYTTPEDATPEPGEDPRVTRAKYFIRDEFLRISTASGDGRHYCYPHFTCAVDTENARRIFNDVTDIIIKMNLRDCGLF

SEQ ID NO: 112 - protein, 263 aa, synthetic construct
  REGION 1..263: note = Mini-Gs/i148
MGHHHHHHENLYFQGNSKTEDQRNEEKAQREANKKIEKQLQKDKQVYRATHRLLLLGADNSGKSTIVKQMRILHGGSGGSGGTSGIFETKFQVDKVNFHMFDVGGQRDERRKWIQCFNDVTAIIFVVDSSDYNRLQEALNLFKSIWNNRWLRTISVILFLNKQDLLAEKVLAGKSKIEDYFPEFARYTTPEDATPEPGEDPRVTRAKYFIRDEFLRISTASGDGRHYCYPHFTCAVDTENARRIFNDVTDIIIKMNLRDCGLF

SEQ ID NO: 113 - protein, 225 aa, synthetic construct
  REGION 1..225: note = Mini-Go112
MGHHHHHHENLYFQGIEKNLKEDGISAAKDVKLLLLGADNSGKSTIVKQMKIIHGGSGGSGGTTGIVETHFTFKNLHFRLFDVGGQRSERKKWIHCFEDVTAIIFCVDLSDYNRMHESLMDFDSICNNKFFIDTSIILFLNKKDLFGEKIKKSPLTICFPEYTGPNTYEDAAAYIQAQFESKNRSPNKEIYCHMTCATDTNNAQVIFDAVTDIIIANNLRGCGLY

SEQ ID NO: 114 - protein, 226 aa, synthetic construct
  REGION 1..226: note = Mini-G128
MGHHHHHHENLYFQGIDALLARERRAVRRLVKILLLGADNSGKSTFLKQMRIIHGGSGGSGGTKGIVEHDFVIKKIPFKMVDVGGQRSQRQKWFQCFDGITSILFMVDSSDYNRLVESMNDFETIVNNKLFFNVSIILFLNKMDLLVEKVKTVSIKKHFPDFRGDPHRLEDVQRYLVQCFDRKRRNRSKPLFHHFTTAIDTENARFIFHAVKDTILQENLKDIMLQ

SEQ ID NO: 115 - DNA, 691 bp, synthetic construct
  misc_feature 1..691: note = Mini-Gt1
  source 1..691: mol_type = other DNA
ccatgggtcaccaccatcaccatcatgaaaatctttatttccagggtctggaaaagaagctgaaagaggacgctgagaaggatgctcgaaccgtgaagctgctgcttctgggtgccgataattccgggaagagcaccatcgtcaagcagatgaagattatccacggtgggagtggcgggagcggaggtaccactggcatcatcgagacgcagttctccttcaaggatctcaacttccggatgttcgatgtgggcgggcagcgctcggagcgcaagaagtggatccactgcttcgagggcgtgacctgcatcatcttcatcgcggacctgagcgattacaaccgcatgcacgagagcctgcacgatttcaacagcatctgcaaccaccgctacttcgccacgacgtccatcgtgctcttccttaacaagaaggacgtcttcttcgagaagatcaagaaggcgcacctcagcatctgtttcccggactacgatggacccaacacctacgaggacgccggcaactacatcaaggtgcagttcctcgagctcaacatgcggcgcgacgtgaaggagatctattcccacatgacgtgcgccaccgacacgcagaacgccaaatttatcttcgacgctgtcaccgacatcatcatcaaggagaacctcaaagactgtggcctcttctaatagctcga

SEQ ID NO: 116 - protein, 226 aa, synthetic construct
  REGION 1..226: note = Mini-Gt1
MGHHHHHHENLYFQGLEKKLKEDAEKDARTVKLLLLGADNSGKSTIVKQMKIIHGGSGGSGGTTGIIETQFSFKDLNFRMFDVGGQRSERKKWIHCFEGVTCIIFIADLSDYNRMHESLHDFNSICNHRYFATTSIVLFLNKKDVFFEKIKKAHLSICFPDYDGPNTYEDAGNYIKVQFLELNMRRDVKEIYSHMTCATDTQNAKFIFDAVTDIIIKENLKDCGLF

SEQ ID NO: 117 - DNA, 671 bp, synthetic construct
  misc_feature 1..671: note = Mini-Gz
  source 1..671: mol_type = other DNA
ccatgggtcaccaccatcaccatcatattgaccgccacctgcgctcagagagccagcggcaacgccgcgaaatcaagctgctcctgctgggcaccgacaactcaggcaagagcaccatcgtcaaacagatgaagatcatccacggagggggcggaggcgggggagggaccacgggcattgtggagaacaagttcaccttcaaggagctcaccttcaagatggtggacgtgggggggcagaggtcagagcgcaaaaagtggatccactgcttcgagggcgtcacagccatcatcttctgtgtggacctcagcgactacagtcggatggcagagagcttgcgcgactttgactccatctgcaacaacaactggttcatcaacacctcactcatcctcttcctgaacaagaaggacctgctggcagagaagatccgccgcatcccgctcaccatctgctttcccgagtacaagggccagaacacgtacgaggaggccgctgtctacatccagcggcagtttgaagacctgaaccgcaacaaggagaccaaggagatctactcccacttcacctgcgccaccgacaccagtaacgcgcagtttatcttcgacgcggtgacagacgtcatcatacagaacaatctcaagtacattggcctttgctgataactcgag

SEQ ID NO: 118 - protein, 219 aa, synthetic construct
  REGION 1..219: note = Mini-Gz
MGHHHHHHIDRHLRSESQRQRREIKLLLLGTDNSGKSTIVKQMKIIHGGGGGGGGTTGIVENKFTFKELTFKMVDVGGQRSERKKWIHCFEGVTAIIFCVDLSDYSRMAESLRDFDSICNNNWFINTSLILFLNKKDLLAEKIRRIPLTICFPEYKGQNTYEEAAVYIQRQFEDLNRNKETKEIYSHFTCATDTSNAQFIFDAVTDVIIQNNLKYIGLC

SEQ ID NO: 119 - DNA, 671 bp, synthetic construct
  misc_feature 1..671: note = Mini-Gq
  source 1..671: mol_type = other DNA
ccatgggtcaccaccatcaccatcatatcgagcggcagctccgcagggacaagcgggacgcccgccgggagctcaagctgctgctgctcgggacagacaacagtggcaagagtacgtttatcaagcagatgagaatcatccacggagggggcggaggcgggggagggaccacagggatcatcgaatacccctttgacttacaaagtgtcattttcagaatggtcgatgtagggggccaaaggtcagagagaagaaaatggatacactgctttgaaaatgtcacctctatcatgtttctagtagaccttagtgactataaccgaatggaggaaagcaaggctgactttagaacaattatcacatacccctggttccagaactcctcggttattctgttcttaaacaagaaagatcttctagaggagaaaatcatgtattcccatctagtcgactacttcccagaatatgatggaccccagagagatgcccaggcagcccgagaattcattctgaagatgttcgtggacctgaacccagacagtgacaaaattatctactcccacttcacgtgcgccacagacaccgagaatgcccgctttatctttgctgccgtcaaggacaccatcctccagttgaacctgaaggagtacaatctggtctaatagctcgag

SEQ ID NO: 120 - protein, 218 aa, synthetic construct
  REGION 1..218: note = Mini-Gq
MGHHHHHHIERQLRRDKRDARRELKLLLLGTDNSGKSTFIKQMRIIHGGGGGGGGTTGIIEYPFDLQSVIFRMVDVGGQRSERRKWIHCFENVTSIMFLVDLSDYNRMEESKADFRTIITYPWFQNSSVILFLNKKDLLEEKIMYSHLVDYFPEYDGPQRDAQAAREFILKMFVDLNPDSDKIIYSHFTCATDTENARFIFAAVKDTILQLNLKEYNL

SEQ ID NO: 121 - DNA, 707 bp, synthetic construct
  misc_feature 1..707: note = Mini-G16
  source 1..707: mol_type = other DNA
ccatgggtcaccaccatcaccatcatatcaacaggatcctcttggagcagaagaagcaggaccgcggggagctgaagctgctgcttttgggcccagacaacagcgggaagagcaccttcatcaagcagatgcggatcatccacggagggggcggaggcgggggagggaccactggcatcaacgagtactgcttctccgtgcagaaaaccaacctgcggatcgtggacgtcgggggccagaagtcagagcgtaagaaatggatccattgtttcgagaacgtgatcgccctcatctacctggccgacctgagtgactacaaccgcatgaaggagagcctcgcagactttgggactatcctggaactaccctggttcaaaagcacatccgtcatcctctttctcaacaaaaccgacatcctggaggagaaaatccccacctcccacctggctacctatttccccagtttccagggccctaagcaggatgctgaggcagccaagaggttcatcctggacatgtacacgaggatgtacaccgggtgcgtggacggccccgagggcagcaagaagggcgcacgatcccgacgcctcttcagccactacacatgtgccacagacacacagaacgcgcgcaagatcttcaaggacgtgcgggactcggtgctcgcccgctacctggacgagatcaacctgctgtaatagctcgag

SEQ ID NO: 122 - protein, 231 aa, synthetic construct
  REGION 1..231: note = Mini-G16
MGHHHHHHINRILLEQKKQDRGELKLLLLGPDNSGKSTFIKQMRIIHGGGGGGGGTTGINEYCFSVQKTNLRIVDVGGQKSERKKWIHCFENVIALIYLADLSDYNRMKESLADFGTILELPWFKSTSVILFLNKTDILEEKIPTSHLATYFPSFQGPKQDAEAAKRFILDMYTRMYTGCVDGPEGSKKGARSRRLFSHYTCATDTQNARKIFKDVRDSVLARYLDEINLL

SEQ ID NO: 123 - protein, 486 aa, synthetic construct
  REGION 1..486: note = GFP-mini-Gs393
MGHHHHHHENLYFQGVSKGEELFTGVVPILVELDGDVNGHKFSVSGEGEGDATYGKLTLKFICTTGKLPVPWPTLVTTLTYGVQCFSRYPDHMKQHDFFKSAMPEGYVQERTIFFKDDGNYKTRAEVKFEGDTLVNRIELKGIDFKEDGNILGHKLEYNYNSHNVYIMADKQKNGIKVNFKIRHNIEDGSVQLADHYQQNTPIGDGPVLLPDNHYLSTQSALSKDPNEKRDHMVLLEFVTAAGITLGMDELYKGGGGSIEKQLQKDKQVYRATHRLLLLGADNSGKSTIVKQMRILHGGSGGSGGTSGIFETKFQVDKVNFHMFDVGGQRDERRKWIQCFNDVTAIIFVVDSSDYNRLQEALNDFKSIWNNRWLRTISVILFLNKQDLLAEKVLAGKSKIEDYFPEFARYTTPEDATPEPGEDPRVTRAKYFIRDEFLRISTASGDGRHYCYPHFTCAVDTENARRIFNDCRDIIQRMHLRQYELL

SEQ ID NO: 124 - protein, 484 aa, synthetic construct
  REGION 1..484: note = GFP-mini-Gi146
MGHHHHHHENLYFQGVSKGEELFTGVVPILVELDGDVNGHKFSVSGEGEGDATYGKLTLKFICTTGKLPVPWPTLVTTLTYGVQCFSRYPDHMKQHDFFKSAMPEGYVQERTIFFKDDGNYKTRAEVKFEGDTLVNRIELKGIDFKEDGNILGHKLEYNYNSHNVYIMADKQKNGIKVNFKIRHNIEDGSVQLADHYQQNTPIGDGPVLLPDNHYLSTQSALSKDPNEKRDHMVLLEFVTAAGITLGMDELYKGGGGSTLSAEDKAAVERSKMIDRNLREDGEKAAREVKLLLLGADNSGKSTIVKQMKIIHGGGGGGGGTTGIVETHFTFKDLHFKMFDVGGQRSERKKWIHCFEDVAAIIFCVDLSDYNRMHESMKLFDSICNNKWFTDTSIILFLNKKDLFEEKIKKSPLTICYQEYAGSNTYEEAAAYIQCQFEDLNKRKDTKEIYTHFTCATDTKNAQFIFDAVTDVIIKNNLKDCGLF

SEQ ID NO: 125 - protein, 486 aa, synthetic construct
  REGION 1..486: note = GFP-mini-Gs/i143
MGHHHHHHENLYFQGVSKGEELFTGVVPILVELDGDVNGHKFSVSGEGEGDATYGKLTLKFICTTGKLPVPWPTLVTTLTYGVQCFSRYPDHMKQHDFFKSAMPEGYVQERTIFFKDDGNYKTRAEVKFEGDTLVNRIELKGIDFKEDGNILGHKLEYNYNSHNVYIMADKQKNGIKVNFKIRHNIEDGSVQLADHYQQNTPIGDGPVLLPDNHYLSTQSALSKDPNEKRDHMVLLEFVTAAGITLGMDELYKGGGGSIEKQLQKDKQVYRATHRLLLLGADNSGKSTIVKQMRILHGGSGGSGGTSGIFETKFQVDKVNFHMFDVGGQRDERRKWIQCFNDVTAIIFVVDSSDYNRLQEALNDFKSIWNNRWLRTISVILFLNKQDLLAEKVLAGKSKIEDYFPEFARYTTPEDATPEPGEDPRVTRAKYFIRDEFLRISTASGDGRHYCYPHFTCAVDTENARRIFNDVTDIIIKMNLRDCGLF

SEQ ID NO: 126 - protein, 468 aa, synthetic construct
  REGION 1..468: note = GFP-mini-Go112
MGHHHHHHENLYFQGVSKGEELFTGVVPILVELDGDVNGHKFSVSGEGEGDATYGKLTLKFICTTGKLPVPWPTLVTTLTYGVQCFSRYPDHMKQHDFFKSAMPEGYVQERTIFFKDDGNYKTRAEVKFEGDTLVNRIELKGIDFKEDGNILGHKLEYNYNSHNVYIMADKQKNGIKVNFKIRHNIEDGSVQLADHYQQNTPIGDGPVLLPDNHYLSTQSALSKDPNEKRDHMVLLEFVTAAGITLGMDELYKGGGGSIEKNLKEDGISAAKDVKLLLLGADNSGKSTIVKQMKIIHGGSGGSGGTTGIVETHFTFKNLHFRLFDVGGQRSERKKWIHCFEDVTAIIFCVDLSDYNRMHESLMDFDSICNNKFFIDTSIILFLNKKDLFGEKIKKSPLTICFPEYTGPNTYEDAAAYIQAQFESKNRSPNKEIYCHMTCATDTNNAQVIFDAVTDIIIANNLRGCGLY

SEQ ID NO: 127 - protein, 469 aa, synthetic construct
  REGION 1..469: note = GFP-mini-G128
MGHHHHHHENLYFQGVSKGEELFTGVVPILVELDGDVNGHKFSVSGEGEGDATYGKLTLKFICTTGKLPVPWPTLVTTLTYGVQCFSRYPDHMKQHDFFKSAMPEGYVQERTIFFKDDGNYKTRAEVKFEGDTLVNRIELKGIDFKEDGNILGHKLEYNYNSHNVYIMADKQKNGIKVNFKIRHNIEDGSVQLADHYQQNTPIGDGPVLLPDNHYLSTQSALSKDPNEKRDHMVLLEFVTAAGITLGMDELYKGGGGSIDALLARERRAVRRLVKILLLGADNSGKSTFLKQMRIIHGGSGGSGGTKGIVEHDFVIKKIPFKMVDVGGQRSQRQKWFQCFDGITSILFMVDSSDYNRLVESMNDFETIVNNKLFFNVSIILFLNKMDLLVEKVKTVSIKKHFPDFRGDPHRLEDVQRYLVQCFDRKRRNRSKPLFHHFTTAIDTENARFIFHAVKDTILQENLKDIMLQ

SEQ ID NO: 128 - protein, 226 aa, synthetic construct
  REGION 1..226: note = mini-Gq
MGHHHHHHENLYFQGIERQLRRDKRDARRELKLLLLGTDNSGKSTFIKQMRIIHGGGGGGGGTTGIIEYPFDLQSVIFRMVDVGGQRSERRKWIHCFENVTSIMFLVDLSDYNRMEESKADFRTIITYPWFQNSSVILFLNKKDLLEEKIMYSHLVDYFPEYDGPQRDAQAAREFILKMFVDLNPDSDKIIYSHFTCATDTENARFIFAAVKDTILQLNLKEYNLV

SEQ ID NO: 129 - protein, 243 aa, synthetic construct; identical to SEQ ID NO: 34
  REGION 1..243: note = mini-Gs

SEQ ID NO: 130 - protein, 243 aa, synthetic construct; identical to SEQ ID NO: 106
  REGION 1..243: note = mini-Gs/q57

SEQ ID NO: 131 - protein, 243 aa, synthetic construct; identical to SEQ ID NO: 107
  REGION 1..243: note = mini-Gs/q58

SEQ ID NO: 132 - protein, 243 aa, synthetic construct; identical to SEQ ID NO: 108
  REGION 1..243: note = mini-Gs/q70

SEQ ID NO: 133 - protein, 243 aa, synthetic construct; identical to SEQ ID NO: 109
  REGION 1..243: note = mini-Gs/q71

SEQ ID NO: 134 - protein, 243 aa, synthetic construct; identical to SEQ ID NO: 34
  REGION 1..243: note = miniGs_393

SEQ ID NO: 135 - protein, 234 aa, synthetic construct
  REGION 1..234: note = miniGi1_46
MGHHHHHHENLYFQGTLSAEDKAAVERSKMIDRNLREDGEKAAREVKLLLLGADNSGKSTIVKQMKIIHGGGGGGGGTTGIVETHFTFKDLHFKMFDVGGQRSERKKWIHCFEDVAAIIFCVDLSDYNRMHESMKLFDSICNNKWFTDTSIILFLNKKDLFEEKIKYQEYAGSNTYEEAAAYIQCQFEDLNKRKDTKEIYTHFTCATDTKNAQFIFDAVTDVIIKNNLKDCGLF

SEQ ID NO: 136 - protein, 243 aa, synthetic construct; identical to SEQ ID NO: 111
  REGION 1..243: note = miniGs/i1_43

SEQ ID NO: 137 - protein, 263 aa, synthetic construct; identical to SEQ ID NO: 112
  REGION 1..263: note = mniGs/i1_48

SEQ ID NO: 138 - protein, 218 aa, synthetic construct
  REGION 1..218: note = miniGo1_12
MGHHHHHHENLYFQGIEKNLKEDGISAAKDVKLLLLGADNSGKSTIVKQMKIIHGGSGGSGGTTGIVETHFTFKNLHFRLFDVGGQRSERKKWIHCFEDVTAIIFCVDLSDYNRMHESLMDFDSICNNKFFIDTSIILFLNKKDLFGEKIKFPEYTGPNTYEDAAAYIQAQFESKNRSPNKEIYCHMTCATDTNNAQVIFDAVTDIIIANNLRGCGLY

SEQ ID NO: 139 - protein, 263 aa, synthetic construct
  REGION 1..263: note = miniGs/o_16
MGHHHHHHENLYFQGNSKTEDQRNEEKAQREANKKIEKQLQKDKQVYRATHRLLLLGADNSGKSTIVKQMRILHGGSGGSGGTSGIFETKFQVDKVNFHMFDVGGQRDERRKWIQCFNDVTAIIFVVDSSDYNRLQEALNLFKSIWNNRWLRTISVILFLNKQDLLAEKVLAGKSKIEDYFPEFARYTTPEDATPEPGEDPRVTRAKYFIRDEFLRISTASGDGRHYCYPHFTCAVDTENARRIFNDVTDIIIAMNLRGCGLY

SEQ ID NO: 140 - protein, 350 aa, synthetic construct
  REGION 1..350: note = G t subunit (chimera 6)
MGAGASAEEKHSRELEKKLKEDAEKDARTVKLLLLGAGESGKSTIVKQMKIIHQDGYSLEECLEFIAIIYGNTLQSILAIVRAMTTLNIQYGDSARQDDARKLMHMADTIEEGTMPKEMSDIIQRLWKDSGIQACFDRASEYQLNDSAGYYLSDLERLVTPGYVPTEQDVLRSRVKTTGIIETQFSFKDLNFRMFDVGGQRSERKKWIHCFEGVTAIIFCVALSDYDLVLAEDEEMNRMHESMKLFDSICNNKWFTDTSIILFLNKKDLFEEKIKKSPLTICYPEYAGSNTYEEAGNYIKVQFLELNMRRDVKEIYSHMTCATDTQNVKFVFDAVTDIIIKENLKDCGLF

SEQ ID NO: 141 - protein, 394 aa, Homo sapiens; identical to SEQ ID NO: 92
  REGION 1..394: note = P63092

SEQ ID NO: 142 - protein, 381 aa, Homo sapiens
  REGION 1..381: note = P38405
MGCLGGNSKTTEDQGVDEKERREANKKIEKQLQKERLAYKATHRLLLLGAGESGKSTIVKQMRILHVNGFNPEEKKQKILDIRKNVKDAIVTIVSAMSTIIPPVPLANPENQFRSDYIKSIAPITDFEYSQEFFDHVKKLWDDEGVKACFERSNEYQLIDCAQYFLERIDSVSLVDYTPTDQDLLRCRVLTSGIFETRFQVDKVNFHMFDVGGQRDERRKWIQCFNDVTAIIYVAACSSYNMVIREDNNTNRLRESLDLFESIWNNRWLRTISIILFLNKQDMLAEKVLAGKSKIEDYFPEYANYTVPEDATPDAGEDPKVTRAKFFIRDLFLRISTATGDGKHYCYPHFTCAVDTENIRRVFNDCRDIIQRMHLKQYELL

SEQ ID NO: 143 - protein, 354 aa, Homo sapiens
  REGION 1..354: note = P63096
MGCTLSAEDKAAVERSKMIDRNLREDGEKAAREVKLLLLGAGESGKSTIVKQMKIIHEAGYSEEECKQYKAVVYSNTIQSIIAIIRAMGRLKIDFGDSARADDARQLFVLAGAAEEGFMTAELAGVIKRLWKDSGVQACFNRSREYQLNDSAAYYLNDLDRIAQPNYIPTQQDVLRTRVKTTGIVETHFTFKDLHFKMFDVGGQRSERKKWIHCFEGVTAIIFCVALSDYDLVLAEDEEMNRMHESMKLFDSICNNKWFTDTSIILFLNKKDLFEEKIKKSPLTICYPEYAGSNTYEEAAAYIQCQFEDLNKRKDTKEIYTHFTCATDTKNVQFVFDAVTDVIIKNNLKDCGLF

SEQ ID NO: 144 - protein, 355 aa, Homo sapiens
  REGION 1..355: note = P04899
MGCTVSAEDKAAAERSKMIDKNLREDGEKAAREVKLLLLGAGESGKSTIVKQMKIIHEDGYSEEECRQYRAVVYSNTIQSIMAIVKAMGNLQIDFADPSRADDARQLFALSCTAEEQGVLPDDLSGVIRRLWADHGVQACFGRSREYQLNDSAAYYLNDLERIAQSDYIPTQQDVLRTRVKTTGIVETHFTFKDLHFKMFDVGGQRSERKKWIHCFEGVTAIIFCVALSAYDLVLAEDEEMNRMHESMKLFDSICNNKWFTDTSIILFLNKKDLFEEKITHSPLTICFPEYTGANKYDEAASYIQSKFEDLNKRKDTKEIYTHFTCATDTKNVQFVFDAVTDVIIKNNLKDCGLF

SEQ ID NO: 145 - protein, 354 aa, Homo sapiens
  REGION 1..354: note = P08754
MGCTLSAEDKAAVERSKMIDRNLREDGEKAAKEVKLLLLGAGESGKSTIVKQMKIIHEDGYSEDECKQYKVVVYSNTIQSIIAIIRAMGRLKIDFGEAARADDARQLFVLAGSAEEGVMTPELAGVIKRLWRDGGVQACFSRSREYQLNDSASYYLNDLDRISQSNYIPTQQDVLRTRVKTTGIVETHFTFKDLYFKMFDVGGQRSERKKWIHCFEGVTAIIFCVALSDYDLVLAEDEEMNRMHESMKLFDSICNNKWFTETSIILFLNKKDLFEEKIKRSPLTICYPEYTGSNTYEEAAAYIQCQFEDLNRRKDTKEIYTHFTCATDTKNVQFVFDAVTDVIIKNNLKECGLY

SEQ ID NO: 146 - protein, 350 aa, Homo sapiens
  REGION 1..350: note = P11488
MGAGASAEEKHSRELEKKLKEDAEKDARTVKLLLLGAGESGKSTIVKQMKIIHQDGYSLEECLEFIAIIYGNTLQSILAIVRAMTTLNIQYGDSARQDDARKLMHMADTIEEGTMPKEMSDIIQRLWKDSGIQACFERASEYQLNDSAGYYLSDLERLVTPGYVPTEQDVLRSRVKTTGIIETQFSFKDLNFRMFDVGGQRSERKKWIHCFEGVTCIIFIAALSAYDMVLVEDDEVNRMHESLHLFNSICNHRYFATTSIVLFLNKKDVFFEKIKKAHLSICFPDYDGPNTYEDAGNYIKVQFLELNMRRDVKEIYSHMTCATDTQNVKFVFDAVTDIIIKENLKDCGLF

SEQ ID NO: 147 - protein, 354 aa, Homo sapiens
  REGION 1..354: note = P19087
MGSGASAEDKELAKRSKELEKKLQEDADKEAKTVKLLLLGAGESGKSTIVKQMKIIHQDGYSPEECLEFKAIIYGNVLQSILAIIRAMTTLGIDYAEPSCADDGRQLNNLADSIEEGTMPPELVEVIRRLWKDGGVQACFERAAEYQLNDSASYYLNQLERITDPEYLPSEQDVLRSRVKTTGIIETKFSVKDLNFRMFDVGGQRSERKKWIHCFEGVTCIIFCAALSAYDMVLVEDDEVNRMHESLHLFNSICNHKFFAATSIVLFLNKKDLFEEKIKKVHLSICFPEYDGNNSYDDAGNYIKSQFLDLNMRKDVKEIYSHMTCATDTQNVKFVFDAVTDIIIKENLKDCGLF

SEQ ID NO: 148 - protein, 354 aa, Homo sapiens
  REGION 1..354: note = A8MTJ3
MGSGISSESKESAKRSKELEKKLQEDAERDARTVKLLLLGAGESGKSTIVKQMKIIHKNGYSEQECMEFKAVIYSNTLQSILAIVKAMTTLGIDYVNPRSAEDQRQLYAMANTLEDGGMTPQLAEVIKRLWRDPGIQACFERASEYQLNDSAAYYLNDLDRITASGYVPNEQDVLHSRVKTTGIIETQFSFKDLHFRMFDVGGQRSERKKWIHCFEGVTCIIFCAALSAYDMVLVEDEEVNRMHESLHLFNSICNHKYFSTTSIVLFLNKKDIFQEKVTKVHLSICFPEYTGPNTFEDAGNYIKNQFLDLNLKKEDKEIYSHMTCATDTQNVKFVFDAVTDIIIKENLKDCGLF

SEQ ID NO: 149 - protein, 354 aa, Homo sapiens
  REGION 1..354: note = P09471
MGCTLSAEERAALERSKAIEKNLKEDGISAAKDVKLLLLGAGESGKSTIVKQMKIIHEDGFSGEDVKQYKPVVYSNTIQSLAAIVRAMDTLGIEYGDKERKADAKMVCDVVSRMEDTEPFSAELLSAMMRLWGDSGIQECFNRSREYQLNDSAKYYLDSLDRIGAADYQPTEQDILRTRVKTTGIVETHFTFKNLHFRLFDVGGQRSERKKWIHCFEDVTAIIFCVALSGYDQVLHEDETTNRMHESLMLFDSICNNKFFIDTSIILFLNKKDLFGEKIKKSPLTICFPEYTGPNTYEDAAAYIQAQFESKNRSPNKEIYCHMTCATDTNNIQVVFDAVTDIIIANNLRGCGLY

SEQ ID NO: 150 - protein, 355 aa, Homo sapiens
  REGION 1..355: note = P19086
MGCRQSSEEKEAARRSRRIDRHLRSESQRQRREIKLLLLGTSNSGKSTIVKQMKIIHSGGFNLEACKEYKPLIIYNAIDSLTRIIRALAALRIDFHNPDRAYDAVQLFALTGPAESKGEITPELLGVMRRLWADPGAQACFSRSSEYHLEDNAAYYLNDLERIAAADYIPTVEDILRSRDMTTGIVENKFTFKELTFKMVDVGGQRSERKKWIHCFEGVTAIIFCVELSGYDLKLYEDNQTSRMAESLRLFDSICNNNWFINTSLILFLNKKDLLAEKIRRIPLTICFPEYKGQNTYEEAAVYIQRQFEDLNRNKETKEIYSHFTCATDTSNIQFVFDAVTDVIIQNNLKYIGLC

SEQ ID NO: 151 - protein, 359 aa, Homo sapiens
  REGION 1..359: note = P50148
MTLESIMACCLSEEAKEARRINDEIERQLRRDKRDARRELKLLLLGTGESGKSTFIKQMRIIHGSGYSDEDKRGFTKLVYQNIFTAMQAMIRAMDTLKIPYKYEHNKAHAQLVREVDVEKVSAFENPYVDAIKSLWNDPGIQECYDRRREYQLSDSTKYYLNDLDRVADPAYLPTQQDVLRVRVPTTGIIEYPFDLQSVIFRMVDVGGQRSERRKWIHCFENVTSIMFLVALSEYDQVLVESDNENRMEESKALFRTIITYPWFQNSSVILFLNKKDLLEEKIMYSHLVDYFPEYDGPQRDAQAAREFILKMFVDLNPDSDKIIYSHFTCATDTENIRFVFAAVKDTILQLNLKEYNLV

SEQ ID NO: 152 - protein, 359 aa, Homo sapiens
  REGION 1..359: note = P29992
MTLESMMACCLSDEVKESKRINAEIEKQLRRDKRDARRELKLLLLGTGESGKSTFIKQMRIIHGAGYSEEDKRGFTKLVYQNIFTAMQAMIRAMETLKILYKYEQNKANALLIREVDVEKVTTFEHQYVSAIKTLWEDPGIQECYDRRREYQLSDSAKYYLTDVDRIATLGYLPTQQDVLRVRVPTTGIIEYPFDLENIIFRMVDVGGQRSERRKWIHCFENVTSIMFLVALSEYDQVLVESDNENRMEESKALFRTIITYPWFQNSSVILFLNKKDLLEDKILYSHLVDYFPEFDGPQRDAQAAREFILKMFVDLNPDSDKIIYSHFTCATDTENIRFVFAAVKDTILQLNLKEYNLV

SEQ ID NO: 153 - protein, 355 aa, Homo sapiens
  REGION 1..355: note = O95837
MAGCCCLSAEEKESQRISAEIERQLRRDKKDARRELKLLLLGTGESGKSTFIKQMRIIHGSGYSDEDRKGFTKLVYQNIFTAMQAMIRAMDTLRIQYVCEQNKENAQIIREVEVDKVSMLSREQVEAIKQLWQDPGIQECYDRRREYQLSDSAKYYLTDIDRIATPSFVPTQQDVLRVRVPTTGIIEYPFDLENIIFRMVDVGGQRSERRKWIHCFESVTSIIFLVALSEYDQVLAECDNENRMEESKALFKTIITYPWFLNSSVILFLNKKDLLEEKIMYSHLISYFPEYTGPKQDVRAARDFILKLYQDQNPDKEKVIYSHFTCATDTDNIRFVFAAVKDTILQLNLREFNLV

SEQ ID NO: 154 - protein, 374 aa, Homo sapiens
  REGION 1..374: note = P30679
MARSLTWRCCPWCLTEDEKAAARVDQEINRILLEQKKQDRGELKLLLLGPGESGKSTFIKQMRIIHGAGYSEEERKGFRPLVYQNIFVSMRAMIEAMERLQIPFSRPESKHHASLVMSQDPYKVTTFEKRYAAAMQWLWRDAGIRAYYERRREFHLLDSAVYYLSHLERITEEGYVPTAQDVLRSRMPTTGINEYCFSVQKTNLRIVDVGGQKSERKKWIHCFENVIALIYLASLSEYDQCLEENNQENRMKESLALFGTILELPWFKSTSVILFLNKTDILEEKIPTSHLATYFPSFQGPKQDAEAAKRFILDMYTRMYTGCVDGPEGSKKGARSRRLFSHYTCATDTQNIRKVFKDVRDSVLARYLDEINLL

SEQ ID NO: 155 - protein, 381 aa, Homo sapiens
  REGION 1..381: note = Q03113
MSGVVRTLSRCLLPAEAGGARERRAGSGARDAEREARRRSRDIDALLARERRAVRRLVKILLLGAGESGKSTFLKQMRIIHGREFDQKALLEFRDTIFDNILKGSRVLVDARDKLGIPWQYSENEKHGMFLMAFENKAGLPVEPATFQLYVPALSALWRDSGIREAFSRRSEFQLGESVKYFLDNLDRIGQLNYFPSKQDILLARKATKGIVEHDFVIKKIPFKMVDVGGQRSQRQKWFQCFDGITSILFMVSSSEYDQVLMEDRRTNRLVESMNIFETIVNNKLFFNVSIILFLNKMDLLVEKVKTVSIKKHFPDFRGDPHRLEDVQRYLVQCFDRKRRNRSKPLFHHFTTAIDTENVRFVFHAVKDTILQENLKDIMLQ

SEQ ID NO: 156 - protein, 377 aa, Homo sapiens
  REGION 1..377: note = Q14344
MADFLPSRSVLSVCFPGCLLTSGEAEQQRKSKEIDKCLSREKTYVKRLVKILLLGAGESGKSTFLKQMRIIHGQDFDQRAREEFRPTIYSNVIKGMRVLVDAREKLHIPWGDNSNQQHGDKMMSFDTRAPMAAQGMVETRVFLQYLPAIRALWADSGIQNAYDRRREFQLGESVKYFLDNLDKLGEPDYIPSQQDILLARRPTKGIHEYDFEIKNVPFKMVDVGGQRSERKRWFECFDSVTSILFLVSSSEFDQVLMEDRLTNRLTESLNIFETIVNNRVFSNVSIILFLNKTDLLEEKVQIVSIKDYFLEFEGDPHCLRDVQKFLVECFRNKRRDQQQKPLYHHFTTAINTENIRLVFRDVKDTILHDNLKQLMLQ

SEQ ID NO: 157 - protein, 5 aa, synthetic construct
  REGION 1..5: note = DDDDK tag
DDDDK

SEQ ID NO: 158 - DNA, 742 bp, synthetic construct
  misc_feature 1..742: note = Mini Gs393 gene sequence
  source 1..742: mol_type = other DNA
ccatgggtcaccaccatcatcaccatgaaaatctttatttccagggtatcgagaagcagctgcagaaggacaagcaggtctaccgggccacgcaccgcctgctgctgctgggtgctgataattctggtaaaagcaccattgtgaagcagatgaggatcctgcatggtgggagtggcgggagcggaggtcttctggaatctttgagaccaagttccaggtggacaaagtcaacttccacatgtttgacgtgggtggccagcgcgatgaacgccgcaagtggatccagtgcttcaacgatgtgactgccatcatcttcgtggtggacagcagcgattacaaccgcctgcaggaggctctgaacgacttcaagagcatctggaacaacagatggctgcgcaccatctctgtgatcctgttcctcaacaagcaagatctgctcgctgagaaagtccttgctgggaaatcgaagattgaggactactttccagaatttgctcgctacactactcctgaggatgctactcccgagcccggagaggacccacgcgtgacccgggccaagtacttcattcgagatgagtttctgaggatcagcactgccagtggagatgggcgtcactactgctaccctcatttcacctgcgctgtggacactgagaacgcccgccgtatcttcaacgactgccgtgacatcattcagcgcatgcaccttcgtcagtacgagctgctctaatagctcgag

SEQ ID NO: 159 - protein, 243 aa, synthetic construct; identical to SEQ ID NO: 34
  REGION 1..243: note = Mini Gs393 protein sequence

SEQ ID NO: 160 - protein, 394 aa, Bos taurus
  REGION 1..394: note = spP04896
MGCLGNSKTEDQRNEEKAQREANKKIEKQLQKDKQVYRATHRLLLLGAGESGKSTIVKQMRILHVNGFNGEGGEEDPQAARSNSDGEKATKVQDIKNNLKEAIETIVAAMSNLVPPVELANPENQFRVDYILSVMNVPDFDFPPEFYEHAKALWEDEGVRACYERSNEYQLIDCAQYFLDKIDVIKQDDYVPSDQDLLRCRVLTSGIFETKFQVDKVNFHMFDVGGQRDERRKWIQCFNDVTAIIFVVASSSYNMVIREDNQTNRLQEALNLFKSIWNNRWLRTISVILFLNKQDLLAEKVLAGKSKIEDYFPEFARYTTPEDATPEPGEDPRVTRAKYFIRDEFLRISTASGDGRHYCYPHFTCAVDTENIRRVFNDCRDIIQRMHLRQYELL

SEQ ID NO: 161 - protein, 229 aa, synthetic construct
  REGION 1..229: note = Mini Gs C
GIEKQLQKDKQVYRATHRLLLLGADNSGKSTIVKQMRIYHGGSGGSGGTSGIFETKFQVDKVNFHMFDVGGQRDERRKWIQCFNDVTAIIFVVDSSDYNRLQEALNDFKSIWNNRWLRTISVILFLNKQDLLAEKVLAGKSKIEDYFPEFARYTTPEDATPEPGEDPRVTRAKYFIRDEFLRISTASGDGRHYCYPHFTCAVDTENARRIFNDCRDIIQRMHLRQYELL

SEQ ID NO: 162 - protein, 229 aa, synthetic construct; identical to SEQ ID NO: 161
  REGION 1..229: note = Mini Gs D

SEQ ID NO: 163 - protein, 413 aa, Homo sapiens
  REGION 1..413: note = adrb2 human
MGQPGNGSAFLLAPNRSHAPDHDVTQQRDEVWVVGMGIVMSLIVLAIVFGNVLVITAIAKFERLQTVTNYFITSLACADLVMGLAVVPFGAAHILMKMWTFGNFWCEFWTSIDVLCVTASIETLCVIAVDRYFAITSPFKYQSLLTKNKARVIILMVWIVSGLTSFLPIQMHWYRATHQEAINCYANETCCDFFTNQAYAIASSIVSFYVPLVIMVFVYSRVFQEAKRQLQKIDKSEGRFHVQNLSQVEQDGRTGHGLRRSSKFCLKEHKALKTLGIIMGTFTLCWLPFFIVNIVHVIQDNLIRKEVYILLNWIGYVNSGFNPLIYCRSPDFRIAFQELLCLRRSSLKAYGNGYSSNGNTGEQSGYHVEQEKENKLLCEDLPGTEDFVGHQGTVPSDNIDSQGRNCSTNDSLL

SEQ ID NO: 164 - protein, 412 aa, Homo sapiens
  REGION 1..412: note = AA2AR human
MPIMGSSVYITVELAIAVLAILGNVLVCWAVWLNSNLQNVTNYFVVSLAAADIAVGVLAIPFAITISTGFCAACHGCLFIACFVLVLTQSSIFSLLAIAIDRYIAIRIPLRYNGLVTGTRAKGIIAICWVLSFAIGLTPMLGWNNCGQPKEGKNHSQGCGEGQVACLFEDVVPMNYMVYFNFFACVLVPLLLMLGVYLRIFLAARRQLKQMESQPLPGERARSTLQKEVHAAKSLAIIVGLFALCWLPLHIINCFTFFCPDCSHAPLWLMYLAIVLSHTNSVVNPFIYAYRIREFRQTFRKIIRSHVLRQQEPFKAAGTSARVLAAHGSDGEQVSLRLNGHPPGVWANGSAPHPERRPNGYALGLVSGGSAQESQGNTGLPDVELLSHELKGVCPEPPGLDDPLAQDGAGVS

SEQ ID NO: 165 - protein, 325 aa, synthetic construct
  REGION 1..325: note = AA2AR human A
MPIMGSSVYITVELAIAVLAILGNVLVCWAVWLNSNLQNVTNYFVVSLAAADIAVGVLAIPFAITISTGFCAACHGCLFIACFVLVLTQSSIFSLLAIAIDRYIAIRIPLRYNGLVTGTRAKGIIAICWVLSFAIGLTPMLGWNNCGQPKEGKAHSQGCGEGQVACLFEDVVPMNYMVYFNFFACVLVPLLLMLGVYLRIFLAARRQLKQMESQPLPGERARSTLQKEVHAAKSLAIIVGLFALCWLPLHIINCFTFFCPDCSHAPLWLMYLAIVLSHTNSVVNPFIYAYRIREFRQTFRKIIRSHVLENLYFQGHHHHHHHHHH

SEQ ID NO: 166 - protein, 325 aa, synthetic construct; identical to SEQ ID NO: 165
  REGION 1..325: note = AA2AR human B